European Patent Specification EP 3 725 807 B1, published November 19, 2025. Title: ANTI-CD47 ANTIBODIES AND METHODS OF USE THEREOF. Applicant: NovImmune S.A. Masternak, Krzysztof Fischer, Nicolas Rousseau, Francois Dheilly, Elie Kosco-Vilbois, Marie. Application PCT/IB2013/003164. The sequence listing filed with the application follows.

SEQUENCE LISTING (287 sequences)

SEQ ID NO: 1 - DNA, 1338 bp, Artificial Sequence
  common heavy chain
gaggtgcagctgttggagtctgggggaggcttggtacagcctggggggtccctgagactctcctgtgcagcctctggattcacctttagcagctatgccatgagctgggtccgccaggctccagggaaggggctggagtgggtctcagctattagtggtagtggtggtagcacatactacgcagactccgtgaagggccggttcaccatctccagagacaattccaagaacacgctgtatctgcaaatgaacagcctgagagccgaggacacggccgtatattactgtgcgaaaagttatggtgcttttgactactggggccagggaaccctggtcacagtctcgagcgcctccaccaagggcccatcggtcttccccctggcaccctcctccaagagcacctctgggggcacagcggccctgggctgcctggtcaaggactacttccccgaaccggtgacagtctcgtggaactcaggagccctgaccagcggcgtgcacaccttcccggctgtcctacagtcctcaggactctactccctcagcagcgtggtgactgtgccctccagcagcttgggcacccagacctacatctgcaacgtgaatcacaagcccagcaacaccaaggtggacaagagagttgagcccaaatcttgtgacaaaactcacacatgcccaccgtgcccagcacctgaactcctggggggaccgtcagtcttcctcttccccccaaaacccaaggacaccctcatgatctcccggacccctgaggtcacatgcgtggtggtggacgtgagccacgaagaccctgaggtcaagttcaactggtacgtggacggcgtggaggtgcataatgccaagacaaagccgcgggaggagcagtacaacagcacgtaccgtgtggtcagcgtcctcaccgtcctgcaccaggactggctgaatggcaaggagtacaagtgcaaggtctccaacaaagccctcccagcccccatcgagaaaaccatctccaaagccaaagggcagccccgagaaccacaggtgtataccctgcccccatctcgggaggagatgaccaagaaccaggtcagcctgacttgcctggtcaaaggcttctatcccagcgacatcgccgtggagtgggagagcaacgggcagccggagaacaactacaagaccacgcctcccgtgctggactccgacggctccttcttcctctatagcaagctcaccgtggacaagtccaggtggcagcaggggaacgtcttctcatgctccgtgatgcatgaggctctgcacaaccactacacgcagaagagcctctccctgtctccgggttaa

SEQ ID NO: 2 - protein, 445 aa, Artificial Sequence
  common heavy chain
EVQLLESGGGLVQPGGSLRLSCAASGFTFSSYAMSWVRQAPGKGLEWVSAISGSGGSTYYADSVKGRFTISRDNSKNTLYLQMNSLRAEDTAVYYCAKSYGAFDYWGQGTLVTVSSASTKGPSVFPLAPSSKSTSGGTAALGCLVKDYFPEPVTVSWNSGALTSGVHTFPAVLQSSGLYSLSSVVTVPSSSLGTQTYICNVNHKPSNTKVDKRVEPKSCDKTHTCPPCPAPELLGGPSVFLFPPKPKDTLMISRTPEVTCVVVDVSHEDPEVKFNWYVDGVEVHNAKTKPREEQYNSTYRVVSVLTVLHQDWLNGKEYKCKVSNKALPAPIEKTISKAKGQPREPQVYTLPPSREEMTKNQVSLTCLVKGFYPSDIAVEWESNGQPENNYKTTPPVLDSDGSFFLYSKLTVDKSRWQQGNVFSCSVMHEALHNHYTQKSLSLSPG

SEQ ID NO: 3 - DNA, 648 bp, Artificial Sequence
  anti-CD47 5A3 kappa light chain
gacatccagatgacccagtctccatcctccctgtctgcatctgtaggagacagagtcaccatcacttgccaggcgagtcaggacattaataagtatttaaattggtatcagcagaaaccagggaaagcccctaagctcctgatctacggtgcatccaggttggaaacaggggtcccatcaaggttcagtggaagtggatctgggacagattttactttcaccatcagcagcctgcagcctgaagatattgcaacatattactgtcagcagaagcacccccgggggccgaggaccttcggccaagggaccaaggtggaaatcaaacgtacggtggctgcaccatctgtcttcatcttcccgccatctgatgagcagttgaaatctggaactgcctctgttgtgtgcctgctgaataacttctatcccagagaggccaaagtacagtggaaggtggataacgccctccaatcgggtaactcccaggagagtgtcacagagcaggacagcaaggacagcacctacagcctcagcagcaccctgacgctgagcaaagcagactacgagaaacacaaagtctacgcctgcgaagtcacccatcagggcctgagctcgcccgtcacaaagagcttcaacaggggagagtgttaa

SEQ ID NO: 4 - protein, 215 aa, Artificial Sequence
  anti-CD47 5A3 kappa light chain
DIQMTQSPSSLSASVGDRVTITCQASQDINKYLNWYQQKPGKAPKLLIYGASRLETGVPSRFSGSGSGTDFTFTISSLQPEDIATYYCQQKHPRGPRTFGQGTKVEIKRTVAAPSVFIFPPSDEQLKSGTASVVCLLNNFYPREAKVQWKVDNALQSGNSQESVTEQDSKDSTYSLSSTLTLSKADYEKHKVYACEVTHQGLSSPVTKSFNRGEC

SEQ ID NO: 5 - DNA, 648 bp, Artificial Sequence
  anti-CD47 5A3-M4 kappa light chain
gacatccagatgacccagtctccatcctccctgtctgcatctgtaggagacagagtcaccatcacttgccaggcgagtcaggacattaataagtatttaaattggtatcagcagaaaccagggaaagcccctaagctcctgatctacggtgcatccaggttggaaacaggggtcccatcaaggttcagtggaagtggatctgggacagattttactttcaccatcagcagcctgcagcctgaagatattgcaacatattactgtcagcagaagcacccccggaacccgaggaccttcggccaagggaccaaggtggaaatcaaacgtacggtggctgcaccatctgtcttcatcttcccgccatctgatgagcagttgaaatctggaactgcctctgttgtgtgcctgctgaataacttctatcccagagaggccaaagtacagtggaaggtggataacgccctccaatcgggtaactcccaggagagtgtcacagagcaggacagcaaggacagcacctacagcctcagcagcaccctgacgctgagcaaagcagactacgagaaacacaaagtctacgcctgcgaagtcacccatcagggcctgagctcgcccgtcacaaagagcttcaacaggggagagtgttaa

SEQ ID NO: 6 - protein, 215 aa, Artificial Sequence
  anti-CD47 5A3-M4 kappa light chain
DIQMTQSPSSLSASVGDRVTITCQASQDINKYLNWYQQKPGKAPKLLIYGASRLETGVPSRFSGSGSGTDFTFTISSLQPEDIATYYCQQKHPRNPRTFGQGTKVEIKRTVAAPSVFIFPPSDEQLKSGTASVVCLLNNFYPREAKVQWKVDNALQSGNSQESVTEQDSKDSTYSLSSTLTLSKADYEKHKVYACEVTHQGLSSPVTKSFNRGEC

SEQ ID NO: 7 - DNA, 648 bp, Artificial Sequence
  anti-CD47 5A3-M3 kappa light chain
gacatccagatgacccagtctccatcctccctgtctgcatctgtaggagacagagtcaccatcacttgccaggcgagtcagtccattagtagttatttaaattggtatcagcagaaaccagggaaagcccctaagctcctgatctacgctgcatcctcgttggaaacaggggtcccatcaaggttcagtggaagtggatctgggacagattttactttcaccatcagcagcctgcagcctgaagatattgcaacatattactgtcagcagaagcacccccgggggccgaggaccttcggccaagggaccaaggtggaaatcaaacgtacggtggctgcaccatctgtcttcatcttcccgccatctgatgagcagttgaaatctggaactgcctctgttgtgtgcctgctgaataacttctatcccagagaggccaaagtacagtggaaggtggataacgccctccaatcgggtaactcccaggagagtgtcacagagcaggacagcaaggacagcacctacagcctcagcagcaccctgacgctgagcaaagcagactacgagaaacacaaagtctacgcctgcgaagtcacccatcagggcctgagctcgcccgtcacaaagagcttcaacaggggagagtgttaa

SEQ ID NO: 8 - protein, 215 aa, Artificial Sequence
  anti-CD47 5A3-M3 kappa light chain
DIQMTQSPSSLSASVGDRVTITCQASQSISSYLNWYQQKPGKAPKLLIYAASSLETGVPSRFSGSGSGTDFTFTISSLQPEDIATYYCQQKHPRGPRTFGQGTKVEIKRTVAAPSVFIFPPSDEQLKSGTASVVCLLNNFYPREAKVQWKVDNALQSGNSQESVTEQDSKDSTYSLSSTLTLSKADYEKHKVYACEVTHQGLSSPVTKSFNRGEC

SEQ ID NO: 9 - DNA, 648 bp, Artificial Sequence
  anti-CD47 5A3-M5 kappa light chain
gacatccagatgacccagtctccatcctccctgtctgcatctgtaggagacagagtcaccatcacttgccaggcgagtcaggacattaataagtatttaaattggtatcagcagaaaccagggaaagcccctaagctcctgatctacggtgcatccaggttggaaacaggggtcccatcaaggttcagtggaagtggatctgggacagattttactttcaccatcagcagcctgcagcctgaagatattgcaacatattactgtcagcagaagcacccccggtacccgaggaccttcggccaagggaccaaggtggaaatcaaacgtacggtggctgcaccatctgtcttcatcttcccgccatctgatgagcagttgaaatctggaactgcctctgttgtgtgcctgctgaataacttctatcccagagaggccaaagtacagtggaaggtggataacgccctccaatcgggtaactcccaggagagtgtcacagagcaggacagcaaggacagcacctacagcctcagcagcaccctgacgctgagcaaagcagactacgagaaacacaaagtctacgcctgcgaagtcacccatcagggcctgagctcgcccgtcacaaagagcttcaacaggggagagtgttaa

SEQ ID NO: 10 - protein, 215 aa, Artificial Sequence
  anti-CD47 5A3-M5 kappa light chain
DIQMTQSPSSLSASVGDRVTITCQASQDINKYLNWYQQKPGKAPKLLIYGASRLETGVPSRFSGSGSGTDFTFTISSLQPEDIATYYCQQKHPRYPRTFGQGTKVEIKRTVAAPSVFIFPPSDEQLKSGTASVVCLLNNFYPREAKVQWKVDNALQSGNSQESVTEQDSKDSTYSLSSTLTLSKADYEKHKVYACEVTHQGLSSPVTKSFNRGEC

SEQ ID NO: 11 - DNA, 648 bp, Artificial Sequence
  anti-CD47 Ke8 kappa light chain
gacatccagatgacccagtctccatcctccctgtctgcatctgtaggagacagagtcaccatcacttgccgggcaagtcagagcattagcagctatttaaattggtatcagcagaaaccagggaaagcccctaagctcctgatctatgctgcatccagtttgcaaagtggggtcccatcaaggttcagtggcagtggatctgggacagatttcactctcaccatcagcagtctgcaacctgaagattttgcaacttactactgtcagcagttccacaagcggcggccgcagaccttcggccaagggaccaaggtggaaatcaaacgtacggtggctgcaccatctgtcttcatcttcccgccatctgatgagcagttgaaatctggaactgcctctgttgtgtgcctgctgaataacttctatcccagagaggccaaagtacagtggaaggtggataacgccctccaatcgggtaactcccaggagagtgtcacagagcaggacagcaaggacagcacctacagcctcagcagcaccctgacgctgagcaaagcagactacgagaaacacaaagtctacgcctgcgaagtcacccatcagggcctgagctcgcccgtcacaaagagcttcaacaggggagagtgttaa

SEQ ID NO: 12 - protein, 215 aa, Artificial Sequence
  anti-CD47 Ke8 kappa light chain
DIQMTQSPSSLSASVGDRVTITCRASQSISSYLNWYQQKPGKAPKLLIYAASSLQSGVPSRFSGSGSGTDFTLTISSLQPEDFATYYCQQFHKRRPQTFGQGTKVEIKRTVAAPSVFIFPPSDEQLKSGTASVVCLLNNFYPREAKVQWKVDNALQSGNSQESVTEQDSKDSTYSLSSTLTLSKADYEKHKVYACEVTHQGLSSPVTKSFNRGEC

SEQ ID NO: 13 - DNA, 648 bp, Artificial Sequence
  anti-CD47 Ke8H5 kappa light chain
gacatccagatgacccagtctccatcctccctgtctgcatctgtaggagacagagtcaccatcacttgccgggcaagtcagagcattgcgaggtatttaaattggtatcagcagaaaccagggaaagcccctaagctcctgatctatgctgcatccagtttgcaaagtggggtcccatcaaggttcagtggcagtggatctgggacagatttcactctcaccatcagcagtctgcaacctgaagattttgcaacttactactgtcagcagttccataagcgtgcgccgcagaccttcggccaagggaccaaggtggaaatcaaacgtacggtggctgcaccatctgtcttcatcttcccgccatctgatgagcagttgaaatctggaactgcctctgttgtgtgcctgctgaataacttctatcccagagaggccaaagtacagtggaaggtggataacgccctccaatcgggtaactcccaggagagtgtcacagagcaggacagcaaggacagcacctacagcctcagcagcaccctgacgctgagcaaagcagactacgagaaacacaaagtctacgcctgcgaagtcacccatcagggcctgagctcgcccgtcacaaagagcttcaacaggggagagtgttaa

SEQ ID NO: 14 - protein, 215 aa, Artificial Sequence
  anti-CD47 Ke8H5 kappa light chain
DIQMTQSPSSLSASVGDRVTITCRASQSIARYLNWYQQKPGKAPKLLIYAASSLQSGVPSRFSGSGSGTDFTLTISSLQPEDFATYYCQQFHKRAPQTFGQGTKVEIKRTVAAPSVFIFPPSDEQLKSGTASVVCLLNNFYPREAKVQWKVDNALQSGNSQESVTEQDSKDSTYSLSSTLTLSKADYEKHKVYACEVTHQGLSSPVTKSFNRGEC

SEQ ID NO: 15 - DNA, 648 bp, Artificial Sequence
  anti-CD47 Ke8B2 kappa light chain
gacatccagatgacccagtctccatcctccctgtctgcatctgtaggagacagagtcaccatcacttgccgggcaagtcagagcattggtaagtatttaaattggtatcagcagaaaccagggaaagcccctaagctcctgatctatgcggcatccaggttgcaaagtggggtcccatcaaggttcagtggcagtggatctgggacagatttcactctcaccatcagcagtctgcaacctgaagattttgcaacttactactgtcagcagaagcacccgcgtgccccgcggaccttcggccaagggaccaaggtggaaatcaaacgtacggtggctgcaccatctgtcttcatcttcccgccatctgatgagcagttgaaatctggaactgcctctgttgtgtgcctgctgaataacttctatcccagagaggccaaagtacagtggaaggtggataacgccctccaatcgggtaactcccaggagagtgtcacagagcaggacagcaaggacagcacctacagcctcagcagcaccctgacgctgagcaaagcagactacgagaaacacaaagtctacgcctgcgaagtcacccatcagggcctgagctcgcccgtcacaaagagcttcaacaggggagagtgttaa

SEQ ID NO: 16 - protein, 215 aa, Artificial Sequence
  anti-CD47 Ke8B2 kappa light chain
DIQMTQSPSSLSASVGDRVTITCRASQSIGKYLNWYQQKPGKAPKLLIYAASRLQSGVPSRFSGSGSGTDFTLTISSLQPEDFATYYCQQKHPRAPRTFGQGTKVEIKRTVAAPSVFIFPPSDEQLKSGTASVVCLLNNFYPREAKVQWKVDNALQSGNSQESVTEQDSKDSTYSLSSTLTLSKADYEKHKVYACEVTHQGLSSPVTKSFNRGEC

SEQ ID NO: 17 - DNA, 648 bp, Artificial Sequence
  anti-CD47 Ke8A2 kappa light chain
gacatccagatgacccagtctccatcctccctgtctgcatctgtaggagacagagtcaccatcacttgccgggcaagtcagagcattgataggtatttaaattggtatcagcagaaaccagggaaagcccctaagctcctgatctatgctgcatccagtttgcaaagtggggtcccatcaaggttcagtggcagtggatctgggacagatttcactctcaccatcagcagtctgcaacctgaagattttgcaacttactactgtcagcagaagcatccccgtgggccgaggaccttcggccaagggaccaaggtggaaatcaaacgtacggtggctgcaccatctgtcttcatcttcccgccatctgatgagcagttgaaatctggaactgcctctgttgtgtgcctgctgaataacttctatcccagagaggccaaagtacagtggaaggtggataacgccctccaatcgggtaactcccaggagagtgtcacagagcaggacagcaaggacagcacctacagcctcagcagcaccctgacgctgagcaaagcagactacgagaaacacaaagtctacgcctgcgaagtcacccatcagggcctgagctcgcccgtcacaaagagcttcaacaggggagagtgttaa

SEQ ID NO: 18 - protein, 215 aa, Artificial Sequence
  anti-CD47 Ke8A2 kappa light chain
DIQMTQSPSSLSASVGDRVTITCRASQSIDRYLNWYQQKPGKAPKLLIYAASSLQSGVPSRFSGSGSGTDFTLTISSLQPEDFATYYCQQKHPRGPRTFGQGTKVEIKRTVAAPSVFIFPPSDEQLKSGTASVVCLLNNFYPREAKVQWKVDNALQSGNSQESVTEQDSKDSTYSLSSTLTLSKADYEKHKVYACEVTHQGLSSPVTKSFNRGEC

SEQ ID NO: 19 - DNA, 648 bp, Artificial Sequence
  anti-CD47 Ke8E8 kappa light chain
gacatccagatgacccagtctccatcctccctgtctgcatctgtaggagacagagtcaccatcacttgccaggcgagtcaggacattaataagtatttaaattggtatcagcagaaaccagggaaagcccctaagctcctgatctatgctgcatccagtttgcaaagtggggtcccatcaaggttcagtggcagtggatctgggacagatttcactctcaccatcagcagtctgcaacctgaagattttgcaacttactactgtcagcagaagcatccccgtggcccgcggaccttcggccaagggaccaaggtggaaatcaaacgtacggtggctgcaccatctgtcttcatcttcccgccatctgatgagcagttgaaatctggaactgcctctgttgtgtgcctgctgaataacttctatcccagagaggccaaagtacagtggaaggtggataacgccctccaatcgggtaactcccaggagagtgtcacagagcaggacagcaaggacagcacctacagcctcagcagcaccctgacgctgagcaaagcagactacgagaaacacaaagtctacgcctgcgaagtcacccatcagggcctgagctcgcccgtcacaaagagcttcaacaggggagagtgttaa

SEQ ID NO: 20 - protein, 215 aa, Artificial Sequence
  anti-CD47 Ke8E8 kappa light chain
DIQMTQSPSSLSASVGDRVTITCQASQDINKYLNWYQQKPGKAPKLLIYAASSLQSGVPSRFSGSGSGTDFTLTISSLQPEDFATYYCQQKHPRGPRTFGQGTKVEIKRTVAAPSVFIFPPSDEQLKSGTASVVCLLNNFYPREAKVQWKVDNALQSGNSQESVTEQDSKDSTYSLSSTLTLSKADYEKHKVYACEVTHQGLSSPVTKSFNRGEC

SEQ ID NO: 21 - DNA, 648 bp, Artificial Sequence
  anti-CD47 Ke8H3 kappa light chain
gacatccagatgacccagtctccatcctccctgtctgcatctgtaggagacagagtcaccatcacttgccgggcaagtcagagcattaataggtatttaaattggtatcagcagaaaccagggaaagcccctaagctcctgatctatgctgcatccaggttgcaaagtggggtcccatcaaggttcagtggcagtggatctgggacagatttcactctcaccatcagcagtctgcaacctgaagattttgcaacttactactgtcagcagaagcatccgcgtgggccgaggaccttcggccaagggaccaaggtggaaatcaaacgtacggtggctgcaccatctgtcttcatcttcccgccatctgatgagcagttgaaatctggaactgcctctgttgtgtgcctgctgaataacttctatcccagagaggccaaagtacagtggaaggtggataacgccctccaatcgggtaactcccaggagagtgtcacagagcaggacagcaaggacagcacctacagcctcagcagcaccctgacgctgagcaaagcagactacgagaaacacaaagtctacgcctgcgaagtcacccatcagggcctgagctcgcccgtcacaaagagcttcaacaggggagagtgttaa

SEQ ID NO: 22 - protein, 215 aa, Artificial Sequence
  anti-CD47 Ke8H3 kappa light chain
DIQMTQSPSSLSASVGDRVTITCRASQSINRYLNWYQQKPGKAPKLLIYAASRLQSGVPSRFSGSGSGTDFTLTISSLQPEDFATYYCQQKHPRGPRTFGQGTKVEIKRTVAAPSVFIFPPSDEQLKSGTASVVCLLNNFYPREAKVQWKVDNALQSGNSQESVTEQDSKDSTYSLSSTLTLSKADYEKHKVYACEVTHQGLSSPVTKSFNRGEC

SEQ ID NO: 23 - DNA, 648 bp, Artificial Sequence
  anti-CD47 Ke8G6 kappa light chain
gacatccagatgacccagtctccatcctccctgtctgcatctgtaggagacagagtcaccatcacttgccgggcaagtcagagcattggtaggtatttaaattggtatcagcagaaaccagggaaagcccctaagctcctgatctatgctgcatccagtttgcaaagtggggtcccatcaaggttcagtggcagtggatctgggacagatttcactctcaccatcagcagtctgcaacctgaagattttgcaacttactactgtcagcagatgcatccgcgtgcgccgaagaccttcggccaagggaccaaggtggaaatcaaacgtacggtggctgcaccatctgtcttcatcttcccgccatctgatgagcagttgaaatctggaactgcctctgttgtgtgcctgctgaataacttctatcccagagaggccaaagtacagtggaaggtggataacgccctccaatcgggtaactcccaggagagtgtcacagagcaggacagcaaggacagcacctacagcctcagcagcaccctgacgctgagcaaagcagactacgagaaacacaaagtctacgcctgcgaagtcacccatcagggcctgagctcgcccgtcacaaagagcttcaacaggggagagtgttaa

SEQ ID NO: 24 - protein, 215 aa, Artificial Sequence
  anti-CD47 Ke8G6 kappa light chain
DIQMTQSPSSLSASVGDRVTITCRASQSIGRYLNWYQQKPGKAPKLLIYAASSLQSGVPSRFSGSGSGTDFTLTISSLQPEDFATYYCQQMHPRAPKTFGQGTKVEIKRTVAAPSVFIFPPSDEQLKSGTASVVCLLNNFYPREAKVQWKVDNALQSGNSQESVTEQDSKDSTYSLSSTLTLSKADYEKHKVYACEVTHQGLSSPVTKSFNRGEC

SEQ ID NO: 25 - DNA, 648 bp, Artificial Sequence
  anti-CD47 Ke8A3 kappa light chain
gacatccagatgacccagtctccatcctccctgtctgcatctgtaggagacagagtcaccatcacttgccgggtaagtcagagcattagtaagtatttaaattggtatcagcagaaaccagggaaagcccctaagctcctgatctatgctgcatccagtttgcaaagtggggtcccatcaaggttcagtggcagtggatctgggacagatttcactctcaccatcagcagtctgcaacctgaagattttgcaacttactactgtcagcagaggcatccccgtgggccgagcaccttcggccaagggaccaaggtggaaatcaaacgtacggtggctgcaccatctgtcttcatcttcccgccatctgatgagcagttgaaatctggaactgcctctgttgtgtgcctgctgaataacttctatcccagagaggccaaagtacagtggaaggtggataacgccctccaatcgggtaactcccaggagagtgtcacagagcaggacagcaaggacagcacctacagcctcagcagcaccctgacgctgagcaaagcagactacgagaaacacaaagtctacgcctgcgaagtcacccatcagggcctgagctcgcccgtcacaaagagcttcaacaggggagagtgttaa

SEQ ID NO: 26 - protein, 215 aa, Artificial Sequence
  anti-CD47 Ke8A3 kappa light chain
DIQMTQSPSSLSASVGDRVTITCRVSQSISKYLNWYQQKPGKAPKLLIYAASSLQSGVPSRFSGSGSGTDFTLTISSLQPEDFATYYCQQRHPRGPSTFGQGTKVEIKRTVAAPSVFIFPPSDEQLKSGTASVVCLLNNFYPREAKVQWKVDNALQSGNSQESVTEQDSKDSTYSLSSTLTLSKADYEKHKVYACEVTHQGLSSPVTKSFNRGEC

SEQ ID NO: 27 - DNA, 648 bp, Artificial Sequence
  anti-CD47 Ke81A3 kappa light chain
gacatccagatgacccagtctccatcctccctgtctgcatctgtaggagacagagtcaccatcacttgccaggcgagtcaggacattaataggtatttaaattggtatcagcagaaaccagggaaagcccctaagctcctgatctatgctgcatccagtttgcaaagtggggtcccatcaaggttcagtggcagtggatctgggacagatttcactctcaccatcagcagtctgcaacctgaagattttgcaacttactactgtcagcagaggcatccgcgtgccccgcggaccttcggccaagggaccaaggtggaaatcaaacgtacggtggctgcaccatctgtcttcatcttcccgccatctgatgagcagttgaaatctggaactgcctctgttgtgtgcctgctgaataacttctatcccagagaggccaaagtacagtggaaggtggataacgccctccaatcgggtaactcccaggagagtgtcacagagcaggacagcaaggacagcacctacagcctcagcagcaccctgacgctgagcaaagcagactacgagaaacacaaagtctacgcctgcgaagtcacccatcagggcctgagctcgcccgtcacaaagagcttcaacaggggagagtgttaa

SEQ ID NO: 28 - protein, 215 aa, Artificial Sequence
  anti-CD47 Ke81A3 kappa light chain
DIQMTQSPSSLSASVGDRVTITCQASQDINRYLNWYQQKPGKAPKLLIYAASSLQSGVPSRFSGSGSGTDFTLTISSLQPEDFATYYCQQRHPRAPRTFGQGTKVEIKRTVAAPSVFIFPPSDEQLKSGTASVVCLLNNFYPREAKVQWKVDNALQSGNSQESVTEQDSKDSTYSLSSTLTLSKADYEKHKVYACEVTHQGLSSPVTKSFNRGEC

SEQ ID NO: 29 - DNA, 648 bp, Artificial Sequence
  anti-CD47 Ke8A8 kappa light chain
gacatccagatgacccagtctccatcctccctgtctgcatctgtaggagacagagtcaccatcacttgccgggcaagtcagagcattagtaagtatttaaattggtatcagcagaaaccagggaaagcccctaagctcctgatctatgctgcatccactttgcaaagtggggtcccatcaaggttcagtggcagtggatctgggacagatttcactctcaccatcagcagtctgcaacctgaagattttgcaacttactactgtcagcagatgcatccgcgtgcgccgaagaccttcggccaagggaccaaggtggaaatcaaacgtacggtggctgcaccatctgtcttcatcttcccgccatctgatgagcagttgaaatctggaactgcctctgttgtgtgcctgctgaataacttctatcccagagaggccaaagtacagtggaaggtggataacgccctccaatcgggtaactcccaggagagtgtcacagagcaggacagcaaggacagcacctacagcctcagcagcaccctgacgctgagcaaagcagactacgagaaacacaaagtctacgcctgcgaagtcacccatcagggcctgagctcgcccgtcacaaagagcttcaacaggggagagtgttaa

SEQ ID NO: 30 - protein, 215 aa, Artificial Sequence
  anti-CD47 Ke8A8 kappa light chain
DIQMTQSPSSLSASVGDRVTITCRASQSISKYLNWYQQKPGKAPKLLIYAASTLQSGVPSRFSGSGSGTDFTLTISSLQPEDFATYYCQQMHPRAPKTFGQGTKVEIKRTVAAPSVFIFPPSDEQLKSGTASVVCLLNNFYPREAKVQWKVDNALQSGNSQESVTEQDSKDSTYSLSSTLTLSKADYEKHKVYACEVTHQGLSSPVTKSFNRGEC

SEQ ID NO: 31 - DNA, 648 bp, Artificial Sequence
  anti-CD47 Ke8C7 kappa light chain
gacatccagatgacccagtctccatcctccctgtctgcatctgtaggagacagagtcaccatcacttgccaggcgagtcaggacattaataggtatttaaattggtatcagcagaaaccagggaaagcccctaagctcctgatctatgctgcatccagtttgcaaagtggggtcccatcaaggttcagtggcagtggatctgggacagatttcactctcaccatcagcagtctgcaacctgaagattttgcaacttactactgtcagcagcgccatccgcgtggcccgaggaccttcggccaagggaccaaggtggaaatcaaacgtacggtggctgcaccatctgtcttcatcttcccgccatctgatgagcagttgaaatctggaactgcctctgttgtgtgcctgctgaataacttctatcccagagaggccaaagtacagtggaaggtggataacgccctccaatcgggtaactcccaggagagtgtcacagagcaggacagcaaggacagcacctacagcctcagcagcaccctgacgctgagcaaagcagactacgagaaacacaaagtctacgcctgcgaagtcacccatcagggcctgagctcgcccgtcacaaagagcttcaacaggggagagtgttaa

SEQ ID NO: 32 - protein, 215 aa, Artificial Sequence
  anti-CD47 Ke8C7 kappa light chain
DIQMTQSPSSLSASVGDRVTITCQASQDINRYLNWYQQKPGKAPKLLIYAASSLQSGVPSRFSGSGSGTDFTLTISSLQPEDFATYYCQQRHPRGPRTFGQGTKVEIKRTVAAPSVFIFPPSDEQLKSGTASVVCLLNNFYPREAKVQWKVDNALQSGNSQESVTEQDSKDSTYSLSSTLTLSKADYEKHKVYACEVTHQGLSSPVTKSFNRGEC

SEQ ID NO: 33 - DNA, 648 bp, Artificial Sequence
  anti-CD47 Ke8G2 kappa light chain
gacatccagatgacccagtctccatcctccctgtctgcatctgtaggagacagagtcaccatcacttgccgggcaagtcagagcattggtaggtatttaaattggtatcagcagaaaccagggaaagcccctaagctcctgatctatgcggcatccaggttgcaaagtggggtcccatcaaggttcagtggcagtggatctgggacagatttcactctcaccatcaacagtctgcaacctgaagattttgcaacttactactgtcagcagaagcatccccgtgcgccgaggaccttcggccaagggaccaaggtggaaatcaaacgtacggtggctgcaccatctgtcttcatcttcccgccatctgatgagcagttgaaatctggaactgcctctgttgtgtgcctgctgaataacttctatcccagagaggccaaagtacagtggaaggtggataacgccctccaatcgggtaactcccaggagagtgtcacagagcaggacagcaaggacagcacctacagcctcagcagcaccctgacgctgagcaaagcagactacgagaaacacaaagtctacgcctgcgaagtcacccatcagggcctgagctcgcccgtcacaaagagcttcaacaggggagagtgttaa

SEQ ID NO: 34 - protein, 215 aa, Artificial Sequence
  anti-CD47 Ke8G2 kappa light chain
DIQMTQSPSSLSASVGDRVTITCRASQSIGRYLNWYQQKPGKAPKLLIYAASRLQSGVPSRFSGSGSGTDFTLTINSLQPEDFATYYCQQKHPRAPRTFGQGTKVEIKRTVAAPSVFIFPPSDEQLKSGTASVVCLLNNFYPREAKVQWKVDNALQSGNSQESVTEQDSKDSTYSLSSTLTLSKADYEKHKVYACEVTHQGLSSPVTKSFNRGEC

SEQ ID NO: 35 - DNA, 648 bp, Artificial Sequence
  anti-CD47 Ke81G9 kappa light chain
gacatccagatgacccagtctccatcctccctgtctgcatctgtaggagacagagtcaccatcacttgccgggcaagtcagagcattgataagtatttaaattggtatcagcagaaaccagggaaagcccctaagctcctgatctatgcggcatccaggttgcaaagtggggtcccatcaaggttcagtggcagtggatctgggacagatttcactctcaccatcagcagtctgcaacctgaagattttgcaacttactactgtcagcagcggcataagcgttccccgcagaccttcggccaagggaccaaggtggaaatcaaacgtacggtggctgcaccatctgtcttcatcttcccgccatctgatgagcagttgaaatctggaactgcctctgttgtgtgcctgctgaataacttctatcccagagaggccaaagtacagtggaaggtggataacgccctccaatcgggtaactcccaggagagtgtcacagagcaggacagcaaggacagcacctacagcctcagcagcaccctgacgctgagcaaagcagactacgagaaacacaaagtctacgcctgcgaagtcacccatcagggcctgagctcgcccgtcacaaagagcttcaacaggggagagtgttaa

SEQ ID NO: 36 - protein, 215 aa, Artificial Sequence
  anti-CD47 Ke81G9 kappa light chain
DIQMTQSPSSLSASVGDRVTITCRASQSIDKYLNWYQQKPGKAPKLLIYAASRLQSGVPSRFSGSGSGTDFTLTISSLQPEDFATYYCQQRHKRSPQTFGQGTKVEIKRTVAAPSVFIFPPSDEQLKSGTASVVCLLNNFYPREAKVQWKVDNALQSGNSQESVTEQDSKDSTYSLSSTLTLSKADYEKHKVYACEVTHQGLSSPVTKSFNRGEC

SEQ ID NO: 37 - DNA, 648 bp, Artificial Sequence
  anti-CD47 Ke8F2 kappa light chain
gacatccagatgacccagtctccatcctccctgtctgcatctgtaggagacagagtcaccatcacttgccgggcaagtcagagcattgataagtatttaaattggtatcagcagaaaccagggaaagcccctaagctcctgatctatgctgcatccagtttgcaaagtggggtcccatcaaggttcagtggcagtggatctgggacagatttcactctcaccatcagcagtctgcaacctgaagattttgcaacttactactgtcagcagaagcatccgcgtgcgccgcggaccttcggccaagggaccaaggtggaaatcaaacgtacggtggctgcaccatctgtcttcatcttcccgccatctgatgagcagttgaaatctggaactgcctctgttgtgtgcctgctgaataacttctatcccagagaggccaaagtacagtggaaggtggataacgccctccaatcgggtaactcccaggagagtgtcacagagcaggacagcaaggacagcacctacagcctcagcagcaccctgacgctgagcaaagcagactacgagaaacacaaagtctacgcctgcgaagtcacccatcagggcctgagctcgcccgtcacaaagagcttcaacaggggagagtgttaa

SEQ ID NO: 38 - protein, 215 aa, Artificial Sequence
  anti-CD47 Ke8F2 kappa light chain
DIQMTQSPSSLSASVGDRVTITCRASQSIDKYLNWYQQKPGKAPKLLIYAASSLQSGVPSRFSGSGSGTDFTLTISSLQPEDFATYYCQQKHPRAPRTFGQGTKVEIKRTVAAPSVFIFPPSDEQLKSGTASVVCLLNNFYPREAKVQWKVDNALQSGNSQESVTEQDSKDSTYSLSSTLTLSKADYEKHKVYACEVTHQGLSSPVTKSFNRGEC

SEQ ID NO: 39 - DNA, 648 bp, Artificial Sequence
  anti-CD47 Ke8B7 kappa light chain
gacatccagatgacccagtctccatcctccctgtctgcatctgtaggagacagagtcaccatcacttgccgggcaagtcagagcattgggaagtatttaaattggtatcagcagaaaccagggaaagcccctaagctcctgatctatgctgcatccagtttgcaaagtggggtcccatcaaggttcagtggcagtggatctgggacagatttcactctcaccatcagcagtctgcaacctgaagattttgcaacttactactgtcagcagatgcatccgcgtagcccgaagaccttcggccaagggaccaaggtggaaatcaaacgtacggtggctgcaccatctgtcttcatcttcccgccatctgatgagcagttgaaatctggaactgcctctgttgtgtgcctgctgaataacttctatcccagagaggccaaagtacagtggaaggtggataacgccctccaatcgggtaactcccaggagagtgtcacagagcaggacagcaaggacagcacctacagcctcagcagcaccctgacgctgagcaaagcagactacgagaaacacaaagtctacgcctgcgaagtcacccatcagggcctgagctcgcccgtcacaaagagcttcaacaggggagagtgttaa

SEQ ID NO: 40 - protein, 215 aa, Artificial Sequence
  anti-CD47 Ke8B7 kappa light chain
DIQMTQSPSSLSASVGDRVTITCRASQSIGKYLNWYQQKPGKAPKLLIYAASSLQSGVPSRFSGSGSGTDFTLTISSLQPEDFATYYCQQMHPRSPKTFGQGTKVEIKRTVAAPSVFIFPPSDEQLKSGTASVVCLLNNFYPREAKVQWKVDNALQSGNSQESVTEQDSKDSTYSLSSTLTLSKADYEKHKVYACEVTHQGLSSPVTKSFNRGEC

SEQ ID NO: 41 - DNA, 648 bp, Artificial Sequence
  anti-CD47 Ke8C4 kappa light chain
gacatccagatgacccagtctccatcctccctgtctgcatctgtaggagacagagtcaccatcacttgccgggcaagtcagagcattagtaggtatttaaattggtatcagcagaaaccagggaaagcccctaagctcctgatctatgctgcatccaatttgcaaagtggggtcccatcaaggttcagtggcagtggatctgggacagatttcactctcaccatcagcagtctgcaacctgaagattttgcaacttactactgtcagcagatgcatccgcgtgggccgaagaccttcggccaagggaccaaggtggaaatcaaacgtacggtggctgcaccatctgtcttcatcttcccgccatctgatgagcagttgaaatctggaactgcctctgttgtgtgcctgctgaataacttctatcccagagaggccaaagtacagtggaaggtggataacgccctccaatcgggtaactcccaggagagtgtcacagagcaggacagcaaggacagcacctacagcctcagcagcaccctgacgctgagcaaagcagactacgagaaacacaaagtctacgcctgcgaagtcacccatcagggcctgagctcgcccgtcacaaagagcttcaacaggggagagtgttaa

SEQ ID NO: 42 - protein, 215 aa, Artificial Sequence
  anti-CD47 Ke8C4 kappa light chain
DIQMTQSPSSLSASVGDRVTITCRASQSISRYLNWYQQKPGKAPKLLIYAASNLQSGVPSRFSGSGSGTDFTLTISSLQPEDFATYYCQQMHPRGPKTFGQGTKVEIKRTVAAPSVFIFPPSDEQLKSGTASVVCLLNNFYPREAKVQWKVDNALQSGNSQESVTEQDSKDSTYSLSSTLTLSKADYEKHKVYACEVTHQGLSSPVTKSFNRGEC

SEQ ID NO: 43 - DNA, 648 bp, Artificial Sequence
  anti-CD47 Ke8F1 kappa light chain
gacatccagatgacccagtctccatcctccctgtctgcatctgtaggagacagagtcaccatcacttgccgggcaagtcagagcattgcttcttatgtaaattggtatcagcagaaaccagggaaagcccctaagctcctgatctatgctgcatccggtttgcaaagtggggtcccatcaaggttcagtggcagtggatctgggacagatttcactctcaccatcagcagtctgcaacctgaagattttgcaacttactactgtcagcagttccataagcgtcggccgcagaccttcggccaagggaccaaggtggaaatcaaacgtacggtggctgcaccatctgtcttcatcttcccgccatctgatgagcagttgaaatctggaactgcctctgttgtgtgcctgctgaataacttctatcccagagaggccaaagtacagtggaaggtggataacgccctccaatcgggtaactcccaggagagtgtcacagagcaggacagcaaggacagcacctacagcctcagcagcaccctgacgctgagcaaagcagactacgagaaacacaaagtctacgcctgcgaagtcacccatcagggcctgagctcgcccgtcacaaagagcttcaacaggggagagtgttaa

SEQ ID NO: 44 - protein, 215 aa, Artificial Sequence
  anti-CD47 Ke8F1 kappa light chain
DIQMTQSPSSLSASVGDRVTITCRASQSIASYVNWYQQKPGKAPKLLIYAASGLQSGVPSRFSGSGSGTDFTLTISSLQPEDFATYYCQQFHKRRPQTFGQGTKVEIKRTVAAPSVFIFPPSDEQLKSGTASVVCLLNNFYPREAKVQWKVDNALQSGNSQESVTEQDSKDSTYSLSSTLTLSKADYEKHKVYACEVTHQGLSSPVTKSFNRGEC

SEQ ID NO: 45 - DNA, 648 bp, Artificial Sequence
  anti-CD47 Ke8G11 kappa light chain
gacatccagatgacccagtctccatcctccctgtctgcatctgtaggagacagagtcaccatcacttgccgggcaagtcagagcattgggaggtatttaaattggtatcagcagaaaccagggaaagcccctaagctcctgatctatgctgcatccagtttgcaaagtggggtcccatcaaggttcagtggcagtggatctgggacagatttcactctcaccatcagcagtctgcaacctgaagattttgcaacttactactgtcagcagatgcatccgcgtgggccgaagaccttcggccaagggaccaaggtggaaatcaaacgtacggtggctgcaccatctgtcttcatcttcccgccatctgatgagcagttgaaatctggaactgcctctgttgtgtgcctgctgaataacttctatcccagagaggccaaagtacagtggaaggtggataacgccctccaatcgggtaactcccaggagagtgtcacagagcaggacagcaaggacagcacctacagcctcagcagcaccctgacgctgagcaaagcagactacgagaaacacaaagtctacgcctgcgaagtcacccatcagggcctgagctcgcccgtcacaaagagcttcaacaggggagagtgttaa

SEQ ID NO: 46 - protein, 215 aa, Artificial Sequence
  anti-CD47 Ke8G11 kappa light chain
DIQMTQSPSSLSASVGDRVTITCRASQSIGRYLNWYQQKPGKAPKLLIYAASSLQSGVPSRFSGSGSGTDFTLTISSLQPEDFATYYCQQMHPRGPKTFGQGTKVEIKRTVAAPSVFIFPPSDEQLKSGTASVVCLLNNFYPREAKVQWKVDNALQSGNSQESVTEQDSKDSTYSLSSTLTLSKADYEKHKVYACEVTHQGLSSPVTKSFNRGEC

SEQ ID NO: 47 - DNA, 648 bp, Artificial Sequence
  anti-CD47 Ke8H6 kappa light chain
gacatccagatgacccagtctccatcctccctgtctgcatctgtaggagacagagtcaccatcacttgccgggcaagtcagagcattagtaagtatttaaattggtatcagcagaaaccagggaaagcccctaagctcctgatctataatgcatccactttgcaaagtggggtcccatcaaggttcagtggcagtggatctgggacagatttcactctcaccatcagcagtctgcaacctgaagattttgcaacttactactgtcagcagaggcatccgcgtgggccgcgcaccttcggccaagggaccaaggtggaaatcaaacgtacggtggctgcaccatctgtcttcatcttcccgccatctgatgagcagttgaaatctggaactgcctctgttgtgtgcctgctgaataacttctatcccagagaggccaaagtacagtggaaggtggataacgccctccaatcgggtaactcccaggagagtgtcacagagcaggacagcaaggacagcacctacagcctcagcagcaccctgacgctgagcaaagcagactacgagaaacacaaagtctacgcctgcgaagtcacccatcagggcctgagctcgcccgtcacaaagagcttcaacaggggagagtgttaa

SEQ ID NO: 48 - protein, 215 aa, Artificial Sequence
  anti-CD47 Ke8H6 kappa light chain
DIQMTQSPSSLSASVGDRVTITCRASQSISKYLNWYQQKPGKAPKLLIYNASTLQSGVPSRFSGSGSGTDFTLTISSLQPEDFATYYCQQRHPRGPRTFGQGTKVEIKRTVAAPSVFIFPPSDEQLKSGTASVVCLLNNFYPREAKVQWKVDNALQSGNSQESVTEQDSKDSTYSLSSTLTLSKADYEKHKVYACEVTHQGLSSPVTKSFNRGEC

SEQ ID NO: 49 - DNA, 648 bp, Artificial Sequence
  anti-CD47 Ke84G9 kappa light chain
gacatccagatgacccagtctccatcctccctgtctgcatctgtaggagacagagtcaccatcacttgccgggcaagtcagagcattagtaagtatttaaattggtatcagcagaaaccagggaaagcccctaagctcctgatctatgctgcatccagtttgcaaagtggggtcccatcaaggttcagtggcagtggatctgggacagatttcactctcaccatcagcagtctgcaacctgaagattttgcaacttactactgtcagcagaagcatccgcgtagcccgcggaccttcggccaagggaccaaggtggaaatcaaacgtacggtggctgcaccatctgtcttcatcttcccgccatctgatgagcagttgaaatctggaactgcctctgttgtgtgcctgctgaataacttctatcccagagaggccaaagtacagtggaaggtggataacgccctccaatcgggtaactcccaggagagtgtcacagagcaggacagcaaggacagcacctacagcctcagcagcaccctgacgctgagcaaagcagactacgagaaacacaaagtctacgcctgcgaagtcacccatcagggcctgagctcgcccgtcacaaagagcttcaacaggggagagtgttaa

SEQ ID NO: 50 - protein, 215 aa, Artificial Sequence
  anti-CD47 Ke84G9 kappa light chain
DIQMTQSPSSLSASVGDRVTITCRASQSISKYLNWYQQKPGKAPKLLIYAASSLQSGVPSRFSGSGSGTDFTLTISSLQPEDFATYYCQQKHPRSPRTFGQGTKVEIKRTVAAPSVFIFPPSDEQLKSGTASVVCLLNNFYPREAKVQWKVDNALQSGNSQESVTEQDSKDSTYSLSSTLTLSKADYEKHKVYACEVTHQGLSSPVTKSFNRGEC

SEQ ID NO: 51 - DNA, 648 bp, Artificial Sequence
  anti-CD47 Ke8A4 kappa light chain
gacatccagatgacccagtctccatcctccctgtctgcatctgtaggagacagagtcaccatcacttgccgggcaagtcagagcattgctaagtatttaaattggtatcagcagaaaccagggaaagcccctaagctcctgatctatgctgcatccagtttgcaaagtggggtcccatcaaggttcagtggcagtggatctgggacagatttcactctcaccatcagcagtctgcaacctgaagattttgcaacttactactgtcagcagttccataagcgtagcccgcagaccttcggccaagggaccaaggtggaaatcaaacgtacggtggctgcaccatctgtcttcatcttcccgccatctgatgagcagttgaaatctggaactgcctctgttgtgtgcctgctgaataacttctatcccagagaggccaaagtacagtggaaggtggataacgccctccaatcgggtaactcccaggagagtgtcacagagcaggacagcaaggacagcacctacagcctcagcagcaccctgacgctgagcaaagcagactacgagaaacacaaagtctacgcctgcgaagtcacccatcagggcctgagctcgcccgtcacaaagagcttcaacaggggagagtgttaa

SEQ ID NO: 52 - protein, 215 aa, Artificial Sequence
  anti-CD47 Ke8A4 kappa light chain
DIQMTQSPSSLSASVGDRVTITCRASQSIAKYLNWYQQKPGKAPKLLIYAASSLQSGVPSRFSGSGSGTDFTLTISSLQPEDFATYYCQQFHKRSPQTFGQGTKVEIKRTVAAPSVFIFPPSDEQLKSGTASVVCLLNNFYPREAKVQWKVDNALQSGNSQESVTEQDSKDSTYSLSSTLTLSKADYEKHKVYACEVTHQGLSSPVTKSFNRGEC

SEQ ID NO: 53 - DNA, 648 bp, Artificial Sequence
  anti-CD47 Ke86G9 kappa light chain
gacatccagatgacccagtctccatcctccctgtctgcatctgtaggagacagagtcaccatcacttgccgggcaagtcagagcattagtaagtatttaaattggtatcagcagaaaccagggaaagcccctaagctcctgatctataatgcatccaatttgcaaagtggggtcccatcaaggttcagtggcagtggatctgggacagatttcactctcaccatcagcagtctgcaacctgaagattttgcaacttactactgtcagcagaggcatccgcgtgggccgaccaccttcggccaagggaccaaggtggaaatcaaacgtacggtggctgcaccatctgtcttcatcttcccgccatctgatgagcagttgaaatctggaactgcctctgttgtgtgcctgctgaataacttctatcccagagaggccaaagtacagtggaaggtggataacgccctccaatcgggtaactcccaggagagtgtcacagagcaggacagcaaggacagcacctacagcctcagcagcaccctgacgctgagcaaagcagactacgagaaacacaaagtctacgcctgcgaagtcacccatcagggcctgagctcgcccgtcacaaagagcttcaacaggggagagtgttaa

SEQ ID NO: 54 - protein, 215 aa, Artificial Sequence
  anti-CD47 Ke86G9 kappa light chain
DIQMTQSPSSLSASVGDRVTITCRASQSISKYLNWYQQKPGKAPKLLIYNASNLQSGVPSRFSGSGSGTDFTLTISSLQPEDFATYYCQQRHPRGPTTFGQGTKVEIKRTVAAPSVFIFPPSDEQLKSGTASVVCLLNNFYPREAKVQWKVDNALQSGNSQESVTEQDSKDSTYSLSSTLTLSKADYEKHKVYACEVTHQGLSSPVTKSFNRGEC

SEQ ID NO: 55 - DNA, 648 bp, Artificial Sequence
  anti-CD47 Ka3 kappa light chain
gacatccagatgacccagtctccatcctccctgtctgcatctgtaggagacagagtcaccatcacttgccgggcaagtcagagcattagcagctatttaaattggtatcagcagaaaccagggaaagcccctaagctcctgatctatgctgcatccagtttgcaaagtggggtcccatcaaggttcagtggcagtggatctgggacagatttcactctcaccatcagcagtctgcaacctgaagattttgcaacttactactgtcagcagatgcacccgcgcgccccgaagaccttcggccaagggaccaaggtggaaatcaaacgtacggtggctgcaccatctgtcttcatcttcccgccatctgatgagcagttgaaatctggaactgcctctgttgtgtgcctgctgaataacttctatcccagagaggccaaagtacagtggaaggtggataacgccctccaatcgggtaactcccaggagagtgtcacagagcaggacagcaaggacagcacctacagcctcagcagcaccctgacgctgagcaaagcagactacgagaaacacaaagtctacgcctgcgaagtcacccatcagggcctgagctcgcccgtcacaaagagcttcaacaggggagagtgttaa

SEQ ID NO: 56 - protein, 215 aa, Artificial Sequence
  anti-CD47 Ka3 kappa light chain
DIQMTQSPSSLSASVGDRVTITCRASQSISSYLNWYQQKPGKAPKLLIYAASSLQSGVPSRFSGSGSGTDFTLTISSLQPEDFATYYCQQMHPRAPKTFGQGTKVEIKRTVAAPSVFIFPPSDEQLKSGTASVVCLLNNFYPREAKVQWKVDNALQSGNSQESVTEQDSKDSTYSLSSTLTLSKADYEKHKVYACEVTHQGLSSPVTKSFNRGEC

SEQ ID NO: 57 - DNA, 648 bp, Artificial Sequence
  anti-CD47 Ka3A2 kappa light chain
gacatccagatgacccagtctccatcctccctgtctgcatctgtaggagacagagtcaccatcacttgccgggcaagtcagagcattagtaagtatttaaattggtatcagcagaaaccagggaaagcccctaagctcctgatctatgctgcatccaggttgcaaagtggggtcccatcaaggttcagtggcagtggatctgggacagatttcactctcaccatcagcagtctgcaacctgaagattttgcaacttactactgtcagcagatgcatcctcgctcgccgaaaaccttcggccaagggaccaaggtggaaatcaaacgtacggtggctgcaccatctgtcttcatcttcccgccatctgatgagcagttgaaatctggaactgcctctgttgtgtgcctgctgaataacttctatcccagagaggccaaagtacagtggaaggtggataacgccctccaatcgggtaactcccaggagagtgtcacagagcaggacagcaaggacagcacctacagcctcagcagcaccctgacgctgagcaaagcagactacgagaaacacaaagtctacgcctgcgaagtcacccatcagggcctgagctcgcccgtcacaaagagcttcaacaggggagagtgttaa

SEQ ID NO: 58 - protein, 215 aa, Artificial Sequence
  anti-CD47 Ka3A2 kappa light chain
DIQMTQSPSSLSASVGDRVTITCRASQSISKYLNWYQQKPGKAPKLLIYAASRLQSGVPSRFSGSGSGTDFTLTISSLQPEDFATYYCQQMHPRSPKTFGQGTKVEIKRTVAAPSVFIFPPSDEQLKSGTASVVCLLNNFYPREAKVQWKVDNALQSGNSQESVTEQDSKDSTYSLSSTLTLSKADYEKHKVYACEVTHQGLSSPVTKSFNRGEC

SEQ ID NO: 59 - DNA, 648 bp, Artificial Sequence
  anti-CD47 Ka3H3 kappa light chain
gacatccagatgacccagtctccatcctccctgtctgcatctgtaggagacagagtcaccatcacttgccaggcgagtcaggacattgctaagtatttaaattggtatcagcagaaaccagggaaagcccctaagctcctgatctatgctgcatccgctttgcaaagtggggtcccatcaaggttcagtggcagtggatctgggacagatttcactctcaccatcagcagtctgcaacctgaagattttgcaacttactactgtcagcagatgcatcctcgctcgccgaaaaccttcggccaagggaccaaggtggaaatcaaacgtacggtggctgcaccatctgtcttcatcttcccgccatctgatgagcagttgaaatctggaactgcctctgttgtgtgcctgctgaataacttctatcccagagaggccaaagtacagtggaaggtggataacgccctccaatcgggtaactcccaggagagtgtcacagagcaggacagcaaggacagcacctacagcctcagcagcaccctgacgctgagcaaagcagactacgagaaacacaaagtctacgcctgcgaagtcacccatcagggcctgagctcgcccgtcacaaagagcttcaacaggggagagtgttaa

SEQ ID NO: 60 - protein, 215 aa, Artificial Sequence
  anti-CD47 Ka3H3 kappa light chain
DIQMTQSPSSLSASVGDRVTITCQASQDIAKYLNWYQQKPGKAPKLLIYAASALQSGVPSRFSGSGSGTDFTLTISSLQPEDFATYYCQQMHPRSPKTFGQGTKVEIKRTVAAPSVFIFPPSDEQLKSGTASVVCLLNNFYPREAKVQWKVDNALQSGNSQESVTEQDSKDSTYSLSSTLTLSKADYEKHKVYACEVTHQGLSSPVTKSFNRGEC

SEQ ID NO: 61 - DNA, 648 bp, Artificial Sequence
  anti-CD47 Ka3A3 kappa light chain
gacatccagatgacccagtctccatcctccctgtctgcatctgtaggagacagagtcaccatcacttgccgggcaagtcagagcattgctagttatttaaattggtatcagcagaaaccagggaaagcccctaagctcctgatctatgcggcatccaggttgcaaagtggggtcccatcaaggttcagtggcagtggatctgggacagatttcactctcaccatcagcagtctgcaacctgaagattttgcaacttactactgtcagcagatgcatcctcgcgcgccgaaaaccttcggccaagggaccaaggtggaaatcaaacgtacggtggctgcaccatctgtcttcatcttcccgccatctgatgagcagttgaaatctggaactgcctctgttgtgtgcctgctgaataacttctatcccagagaggccaaagtacagtggaaggtggataacgccctccaatcgggtaactcccaggagagtgtcacagagcaggacagcaaggacagcacctacagcctcagcagcaccctgacgctgagcaaagcagactacgagaaacacaaagtctacgcctgcgaagtcacccatcagggcctgagctcgcccgtcacaaagagcttcaacaggggagagtgttaa

SEQ ID NO: 62 - protein, 215 aa, Artificial Sequence
  anti-CD47 Ka3A3 kappa light chain
DIQMTQSPSSLSASVGDRVTITCRASQSIASYLNWYQQKPGKAPKLLIYAASRLQSGVPSRFSGSGSGTDFTLTISSLQPEDFATYYCQQMHPRAPKTFGQGTKVEIKRTVAAPSVFIFPPSDEQLKSGTASVVCLLNNFYPREAKVQWKVDNALQSGNSQESVTEQDSKDSTYSLSSTLTLSKADYEKHKVYACEVTHQGLSSPVTKSFNRGEC

SEQ ID NO: 63 - DNA, 648 bp, Artificial Sequence
  anti-CD47 Ka3H8 kappa light chain
gacatccagatgacccagtctccatcctccctgtctgcatctgtaggagacagagtcaccatcacttgccgggcaagtcagagcattgcgagttatttaaattggtatcagcagaaaccagggaaagcccctaagctcctgatctatgcggcatccaggttgcaaagtggggtcccatcaaggttcagtggcagtggatctgggacagatttcactctcaccatcagcagtctgcaacctgaagattttgcaacttactactgtcagcagatgcatcctcgctcgccgaaaaccttcggccaagggaccaaggtggaaatcaaacgtacggtggctgcaccatctgtcttcatcttcccgccatctgatgagcagttgaaatctggaactgcctctgttgtgtgcctgctgaataacttctatcccagagaggccaaagtacagtggaaggtggataacgccctccaatcgggtaactcccaggagagtgtcacagagcaggacagcaaggacagcacctacagcctcagcagcaccctgacgctgagcaaagcagactacgagaaacacaaagtctacgcctgcgaagtcacccatcagggcctgagctcgcccgtcacaaagagcttcaacaggggagagtgttaa

SEQ ID NO: 64 - protein, 215 aa, Artificial Sequence
  anti-CD47 Ka3H8 kappa light chain
DIQMTQSPSSLSASVGDRVTITCRASQSIASYLNWYQQKPGKAPKLLIYAASRLQSGVPSRFSGSGSGTDFTLTISSLQPEDFATYYCQQMHPRSPKTFGQGTKVEIKRTVAAPSVFIFPPSDEQLKSGTASVVCLLNNFYPREAKVQWKVDNALQSGNSQESVTEQDSKDSTYSLSSTLTLSKADYEKHKVYACEVTHQGLSSPVTKSFNRGEC

SEQ ID NO: 65 - DNA, 648 bp, Artificial Sequence
  anti-CD47 Ka3B2 kappa light chain
gacatccagatgacccagtctccatcctccctgtctgcatctgtaggagacagagtcaccatcacttgccgggcaagtcagaacattggtaagtatttaaattggtatcagcagaaaccagggaaagcccctaagctcctgatctatagtgcatccaggttgcaaagtggggtcccatcaaggttcagtggcagtggatctgggacagatttcactctcaccatcagcagtctgcaacctgaagattttgcaacttactactgtcagcagatgcatcctcgcgcgccgaaaaccttcggccaagggaccaaggtggaaatcaaacgtacggtggctgcaccatctgtcttcatcttcccgccatctgatgagcagttgaaatctggaactgcctctgttgtgtgcctgctgaataacttctatcccagagaggccaaagtacagtggaaggtggataacgccctccaatcgggtaactcccaggagagtgtcacagagcaggacagcaaggacagcacctacagcctcagcagcaccctgacgctgagcaaagcagactacgagaaacacaaagtctacgcctgcgaagtcacccatcagggcctgagctcgcccgtcacaaagagcttcaacaggggagagtgttaa

SEQ ID NO: 66 - protein, 215 aa, Artificial Sequence
  anti-CD47 Ka3B2 kappa light chain
DIQMTQSPSSLSASVGDRVTITCRASQNIGKYLNWYQQKPGKAPKLLIYSASRLQSGVPSRFSGSGSGTDFTLTISSLQPEDFATYYCQQMHPRAPKTFGQGTKVEIKRTVAAPSVFIFPPSDEQLKSGTASVVCLLNNFYPREAKVQWKVDNALQSGNSQESVTEQDSKDSTYSLSSTLTLSKADYEKHKVYACEVTHQGLSSPVTKSFNRGEC

SEQ ID NO: 67 - DNA, 648 bp, Artificial Sequence
  anti-CD47 Ka3C5 kappa light chain
gacatccagatgacccagtctccatcctccctgtctgcatctgtaggagacagagtcaccatcacttgccgggcaagtcagagcattagtaggtatttaaattggtatcagcagaaaccagggaaagcccctaagctcctgatctattctgcatcctctttgcaaagtggggtcccatcaaggttcagtggcagtggatctgggacagatttcactctcaccatcagcagtctgcaacctgaagattttgcaacttactactgtcagcagatgcatcctcgcgccccgaaaaccttcggccaagggaccaaggtggaaatcaaacgtacggtggctgcaccatctgtcttcatcttcccgccatctgatgagcagttgaaatctggaactgcctctgttgtgtgcctgctgaataacttctatcccagagaggccaaagtacagtggaaggtggataacgccctccaatcgggtaactcccaggagagtgtcacagagcaggacagcaaggacagcacctacagcctcagcagcaccctgacgctgagcaaagcagactacgagaaacacaaagtctacgcctgcgaagtcacccatcagggcctgagctcgcccgtcacaaagagcttcaacaggggagagtgttaa

SEQ ID NO: 68 - protein, 215 aa, Artificial Sequence
  anti-CD47 Ka3C5 kappa light chain
DIQMTQSPSSLSASVGDRVTITCRASQSISRYLNWYQQKPGKAPKLLIYSASSLQSGVPSRFSGSGSGTDFTLTISSLQPEDFATYYCQQMHPRAPKTFGQGTKVEIKRTVAAPSVFIFPPSDEQLKSGTASVVCLLNNFYPREAKVQWKVDNALQSGNSQESVTEQDSKDSTYSLSSTLTLSKADYEKHKVYACEVTHQGLSSPVTKSFNRGEC

SEQ ID NO: 69 - DNA, 648 bp, Artificial Sequence
  anti-CD47 Ka3G2 kappa light chain
gacatccagatgacccagtctccatcctccctgtctgcatctgtaggagacagagtcaccatcacttgccgggcaagtcagagcattgataagtatttaaattggtatcagcagaaaccagggaaagcccctaagctcctgatctatgctgcatccaggttgcaaagtggggtcccatcaaggttcagtggcagtggatctgggacagatttcactctcaccatcagcagtctgcaacctgaagattttgcaacttactactgtcagcagatgcatcctcgcgggccgaaaaccttcggccaagggaccaaggtggaaatcaaacgtacggtggctgcaccatctgtcttcatcttcccgccatctgatgagcagttgaaatctggaactgcctctgttgtgtgcctgctgaataacttctatcccagagaggccaaagtacagtggaaggtggataacgccctccaatcgggtaactcccaggagagtgtcacagagcaggacagcaaggacagcacctacagcctcagcagcaccctgacgctgagcaaagcagactacgagaaacacaaagtctacgcctgcgaagtcacccatcagggcctgagctcgcccgtcacaaagagcttcaacaggggagagtgttaa

SEQ ID NO: 70 - protein, 215 aa, Artificial Sequence
  anti-CD47 Ka3G2 kappa light chain
DIQMTQSPSSLSASVGDRVTITCRASQSIDKYLNWYQQKPGKAPKLLIYAASRLQSGVPSRFSGSGSGTDFTLTISSLQPEDFATYYCQQMHPRGPKTFGQGTKVEIKRTVAAPSVFIFPPSDEQLKSGTASVVCLLNNFYPREAKVQWKVDNALQSGNSQESVTEQDSKDSTYSLSSTLTLSKADYEKHKVYACEVTHQGLSSPVTKSFNRGEC

SEQ ID NO: 71 - DNA, 648 bp, Artificial Sequence
  anti-CD47 Ka3D3 kappa light chain
gacatccagatgacccagtctccatcctccctgtctgcatctgtaggagacagagtcaccatcacttgccgggcaagtcagagcattggtaagtatttaaattggtatcagcagaaaccagggaaagcccctaagctcctgatctatgctgcatccaggttgcaaagtggggtcccatcaaggttcagtggcagtggatctgggacagatttcactctcaccatcagcagtctgcaacctgaagattttgcaacttactactgtcagcagatgcatcctcgcgcgccgaaaaccttcggccaagggaccaaggtggaaatcaaacgtacggtggctgcaccatctgtcttcatcttcccgccatctgatgagcagttgaaatctggaactgcctctgttgtgtgcctgctgaataacttctatcccagagaggccaaagtacagtggaaggtggataacgccctccaatcgggtaactcccaggagagtgtcacagagcaggacagcaaggacagcacctacagcctcagcagcaccctgacgctgagcaaagcagactacgagaaacacaaagtctacgcctgcgaagtcacccatcagggcctgagctcgcccgtcacaaagagcttcaacaggggagagtgttaa

SEQ ID NO: 72 - protein, 215 aa, Artificial Sequence
  anti-CD47 Ka3D3 kappa light chain
DIQMTQSPSSLSASVGDRVTITCRASQSIGKYLNWYQQKPGKAPKLLIYAASRLQSGVPSRFSGSGSGTDFTLTISSLQPEDFATYYCQQMHPRAPKTFGQGTKVEIKRTVAAPSVFIFPPSDEQLKSGTASVVCLLNNFYPREAKVQWKVDNALQSGNSQESVTEQDSKDSTYSLSSTLTLSKADYEKHKVYACEVTHQGLSSPVTKSFNRGEC

SEQ ID NO: 73 - DNA, 654 bp, Artificial Sequence
  anti-CD47 Kc4 kappa light chain
cagtctgccctgactcagcctgcctccgtgtctgggtctcctggacagtcgatcaccatctcctgcactggaaccagcagtgacgttggtggttataactatgtctcctggtaccaacagcacccaggcaaagcccccaaactcatgatttatgaggtcagtaatcggccctcaggggtttctaatcgcttctctggctccaagtctggcaacacggcctccctgaccatctctgggctccaggctgaggacgaggctgattattactgcagctcatatgattggtggttccgccccaaggtgttcggcggagggaccaagctgaccgtcctaggtcagcccaaggctgccccctcggtcactctgttcccgccctcctctgaggagcttcaagccaacaaggccacactggtgtgtctcataagtgacttctacccgggagccgtgacagtggcttggaaagcagatagcagccccgtcaaggcgggagtggagaccaccacaccctccaaacaaagcaacaacaagtacgcggccagcagctatctgagcctgacgcctgagcagtggaagtcccacagaagctacagctgccaggtcacgcatgaagggagcaccgtggagaagacagtggcccctacagaatgttcataa

SEQ ID NO: 74 - protein, 217 aa, Artificial Sequence
  anti-CD47 Kc4 kappa light chain
QSALTQPASVSGSPGQSITISCTGTSSDVGGYNYVSWYQQHPGKAPKLMIYEVSNRPSGVSNRFSGSKSGNTASLTISGLQAEDEADYYCSSYDWWFRPKVFGGGTKLTVLGQPKAAPSVTLFPPSSEELQANKATLVCLISDFYPGAVTVAWKADSSPVKAGVETTTPSKQSNNKYAASSYLSLTPEQWKSHRSYSCQVTHEGSTVEKTVAPTECS

SEQ ID NO: 75 - DNA, 654 bp, Artificial Sequence
  anti-CD47 Kc4G11 kappa light chain
cagtctgccctgactcagcctgcctccgtgtctgggtctcctggacagtcgatcaccatctcctgcactggaaccagcagtgacgttgggaaggcgaactatgtctcctggtaccaacagcacccaggcaaagcccccaaactcatgatttataaggatagtgatcggccctcaggggtttctaatcgcttctctggctccaagtctggcaacacggcctccctgaccatctctgggctccaggctgaggacgaggctgattattactgcagctcatatgattggtggttccgccccaaggtgttcggcggagggaccaagctgaccgtcctaggtcagcccaaggctgccccctcggtcactctgttcccgccctcctctgaggagcttcaagccaacaaggccacactggtgtgtctcataagtgacttctacccgggagccgtgacagtggcttggaaagcagatagcagccccgtcaaggcgggagtggagaccaccacaccctccaaacaaagcaacaacaagtacgcggccagcagctatctgagcctgacgcctgagcagtggaagtcccacagaagctacagctgccaggtcacgcatgaagggagcaccgtggagaagacagtggcccctacagaatgttcataa

SEQ ID NO: 76 - protein, 217 aa, Artificial Sequence
  anti-CD47 Kc4G11 kappa light chain
QSALTQPASVSGSPGQSITISCTGTSSDVGKANYVSWYQQHPGKAPKLMIYKDSDRPSGVSNRFSGSKSGNTASLTISGLQAEDEADYYCSSYDWWFRPKVFGGGTKLTVLGQPKAAPSVTLFPPSSEELQANKATLVCLISDFYPGAVTVAWKADSSPVKAGVETTTPSKQSNNKYAASSYLSLTPEQWKSHRSYSCQVTHEGSTVEKTVAPTECS

SEQ ID NO: 77 - DNA, 654 bp, Artificial Sequence
  anti-CD47 Kc4C11 kappa light chain
cagtctgccctgactcagcctgcctccgtgtctgggtctcctggacagtcgatcaccatctcctgcactggaaccagcagtgacgttagggggaataactatgtctcctggtaccaacagcacccaggcaaagcccccaaactcatgatttatgagaatagtaagcggccctcaggggtttctaatcgcttctctggctccaagtctggcaacacggcctccctgaccatctctgggctccaggctgaggacgaggctgattattactgcagctcatatgattggtggttccgccccaaggtgttcggcggagggaccaagctgaccgtcctaggtcagcccaaggctgccccctcggtcactctgttcccgccctcctctgaggagcttcaagccaacaaggccacactggtgtgtctcataagtgacttctacccgggagccgtgacagtggcttggaaagcagatagcagccccgtcaaggcgggagtggagaccaccacaccctccaaacaaagcaacaacaagtacgcggccagcagctatctgagcctgacgcctgagcagtggaagtcccacagaagctacagctgccaggtcacgcatgaagggagcaccgtggagaagacagtggcccctacagaatgttcataa

SEQ ID NO: 78 - protein, 217 aa, Artificial Sequence
  anti-CD47 Kc4C11 kappa light chain
QSALTQPASVSGSPGQSITISCTGTSSDVRGNNYVSWYQQHPGKAPKLMIYENSKRPSGVSNRFSGSKSGNTASLTISGLQAEDEADYYCSSYDWWFRPKVFGGGTKLTVLGQPKAAPSVTLFPPSSEELQANKATLVCLISDFYPGAVTVAWKADSSPVKAGVETTTPSKQSNNKYAASSYLSLTPEQWKSHRSYSCQVTHEGSTVEKTVAPTECS

SEQ ID NO: 79 - DNA, 654 bp, Artificial Sequence
  anti-CD47 Kc4A1 kappa light chain
cagtctgccctgactcagcctgcctccgtgtctgggtctcctggacagtcgatcaccatctcctgcactggaaccagcagtgacgttagtgcgaggaactatgtctcctggtaccaacagcacccaggcaaagcccccaaactcatgatttatgagagtagtaagcggccctcaggggtttctaatcgcttctctggctccaagtctggcaacacggcctccctgaccatctctgggctccaggctgaggacgaggctgattattactgcagctcatatgattggtggttccgccccaaggtgttcggcggagggaccaagctgaccgtcctaggtcagcccaaggctgccccctcggtcactctgttcccgccctcctctgaggagcttcaagccaacaaggccacactggtgtgtctcataagtgacttctacccgggagccgtgacagtggcttggaaagcagatagcagccccgtcaaggcgggagtggagaccaccacaccctccaaacaaagcaacaacaagtacgcggccagcagctatctgagcctgacgcctgagcagtggaagtcccacagaagctacagctgccaggtcacgcatgaagggagcaccgtggagaagacagtggcccctacagaatgttcataa

SEQ ID NO: 80 - protein, 217 aa, Artificial Sequence
  anti-CD47 Kc4A1 kappa light chain
QSALTQPASVSGSPGQSITISCTGTSSDVSARNYVSWYQQHPGKAPKLMIYESSKRPSGVSNRFSGSKSGNTASLTISGLQAEDEADYYCSSYDWWFRPKVFGGGTKLTVLGQPKAAPSVTLFPPSSEELQANKATLVCLISDFYPGAVTVAWKADSSPVKAGVETTTPSKQSNNKYAASSYLSLTPEQWKSHRSYSCQVTHEGSTVEKTVAPTECS

SEQ ID NO: 81 - DNA, 654 bp, Artificial Sequence
  anti-CD47 Kc4A4 kappa light chain
cagtctgccctgactcagcctgcctccgtgtctgggtctcctggacagtcgatcaccatctcctgcactagaaccagcagtgacgttaataatactaactatgtctcctggtaccaacagcacccaggcaaagcccccaaactcatgatttataagactagtggtcggccctcaggggtttctaatcgcttctctggctccaagtctggcaacacggcctccctgaccatctctgggctccaggctgaggacgaggctgattattactgcagctcatatgattggtggttccgccccaaggtgttcggcggagggaccaagctgaccgtcctaggtcagcccaaggctgccccctcggtcactctgttcccgccctcctctgaggagcttcaagccaacaaggccacactggtgtgtctcataagtgacttctacccgggagccgtgacagtggcttggaaagcagatagcagccccgtcaaggcgggagtggagaccaccacaccctccaaacaaagcaacaacaagtacgcggccagcagctatctgagcctgacgcctgagcagtggaagtcccacagaagctacagctgccaggtcacgcatgaagggagcaccgtggagaagacagtggcccctacagaatgttcataa

SEQ ID NO: 82 - protein, 217 aa, Artificial Sequence
  anti-CD47 Kc4A4 kappa light chain
QSALTQPASVSGSPGQSITISCTRTSSDVNNTNYVSWYQQHPGKAPKLMIYKTSGRPSGVSNRFSGSKSGNTASLTISGLQAEDEADYYCSSYDWWFRPKVFGGGTKLTVLGQPKAAPSVTLFPPSSEELQANKATLVCLISDFYPGAVTVAWKADSSPVKAGVETTTPSKQSNNKYAASSYLSLTPEQWKSHRSYSCQVTHEGSTVEKTVAPTECS

SEQ ID NO: 83 - DNA, 654 bp, Artificial Sequence
  anti-CD47 Kc4E10 kappa light chain
cagtctgccctgactcagcctgcctccgtgtctgggtctcctggacagtcgatcaccatctcctgcactggaaccagcagtgacgttaattctgctaactatgtctcctggtaccaacagcacccaggcaaagcccccaaactcatgatttataagagtagtagtcggccctcaggggtttctaatcgcttctctggctccaagtctggcaacacggcctccctgaccatctctgggctccaggctgaggacgaggctgattattactgcagctcatatgattggtggttccgccccaaggtgttcggcggagggaccaagctgaccgtcctaggtcagcccaaggctgccccctcggtcactctgttcccgccctcctctgaggagcttcaagccaacaaggccacactggtgtgtctcataagtgacttctacccgggagccgtgacagtggcttggaaagcagatagcagccccgtcaaggcgggagtggagaccaccacaccctccaaacaaagcaacaacaagtacgcggccagcagctatctgagcctgacgcctgagcagtggaagtcccacagaagctacagctgccaggtcacgcatgaagggagcaccgtggagaagacagtggcccctacagaatgttcataa

SEQ ID NO: 84 - protein, 217 aa, Artificial Sequence
  anti-CD47 Kc4E10 kappa light chain
QSALTQPASVSGSPGQSITISCTGTSSDVNSANYVSWYQQHPGKAPKLMIYKSSSRPSGVSNRFSGSKSGNTASLTISGLQAEDEADYYCSSYDWWFRPKVFGGGTKLTVLGQPKAAPSVTLFPPSSEELQANKATLVCLISDFYPGAVTVAWKADSSPVKAGVETTTPSKQSNNKYAASSYLSLTPEQWKSHRSYSCQVTHEGSTVEKTVAPTECS

SEQ ID NO: 85 - DNA, 654 bp, Artificial Sequence
  anti-CD47 Kc4G9 kappa light chain
cagtctgccctgactcagcctgcctccgtgtccgggtctcctggacagtcgatcaccatctcctgcactggaaccagcagtgacgttgagaggaagaactatgtctcctggtaccaacagcacccaggcaaagcccccaaactcatgatttataagaatagtactcggccctcaggggtttctaatcgcttctctggctccaagtctggcaacacggcctccctgaccatctctgggctccaggctgaggacgaggctgattattactgcagctcatatgattggtggttccgccccaaggtgttcggcggagggaccaagctgaccgtcctaggtcagcccaaggctgccccctcggtcactctgttcccgccctcctctgaggagcttcaagccaacaaggccacactggtgtgtctcataagtgacttctacccgggagccgtgacagtggcttggaaagcagatagcagccccgtcaaggcgggagtggagaccaccacaccctccaaacaaagcaacaacaagtacgcggccagcagctatctgagcctgacgcctgagcagtggaagtcccacagaagctacagctgccaggtcacgcatgaagggagcaccgtggagaagacagtggcccctacagaatgttcataa

SEQ ID NO: 86 - protein, 217 aa, Artificial Sequence
  anti-CD47 Kc4G9 kappa light chain
QSALTQPASVSGSPGQSITISCTGTSSDVERKNYVSWYQQHPGKAPKLMIYKNSTRPSGVSNRFSGSKSGNTASLTISGLQAEDEADYYCSSYDWWFRPKVFGGGTKLTVLGQPKAAPSVTLFPPSSEELQANKATLVCLISDFYPGAVTVAWKADSSPVKAGVETTTPSKQSNNKYAASSYLSLTPEQWKSHRSYSCQVTHEGSTVEKTVAPTECS

SEQ ID NO: 87 - DNA, 654 bp, Artificial Sequence
  anti-CD47 Kc4C3 kappa light chain
cagtctgccctgactcagcctgcctccgtgtctgggtctcctggacagtcgatcaccatctcctgcactggaaccagcagtgacgttagggcggctaactatgtctcctggtaccaacagcacccaggcaaagcccccaaactcatgatttataagaatagtactcggccctcaggggtttctaatcgcttctctggctccaagtctggcaacacggcctccctgaccatctctgggctccaggctgaggacgaggctgattattactgcagctcatatgattggtggttccgccccaaggtgttcggcggagggaccaagctgaccgtcctaggtcagcccaaggctgccccctcggtcactctgttcccgccctcctctgaggagcttcaagccaacaaggccacactggtgtgtctcataagtgacttctacccgggagccgtgacagtggcttggaaagcagatagcagccccgtcaaggcgggagtggagaccaccacaccctccaaacaaagcaacaacaagtacgcggccagcagctatctgagcctgacgcctgagcagtggaagtcccacagaagctacagctgccaggtcacgcatgaagggagcaccgtggagaagacagtggcccctacagaatgttcataa

SEQ ID NO: 88 - protein, 217 aa, Artificial Sequence
  anti-CD47 Kc4C3 kappa light chain
QSALTQPASVSGSPGQSITISCTGTSSDVRAANYVSWYQQHPGKAPKLMIYKNSTRPSGVSNRFSGSKSGNTASLTISGLQAEDEADYYCSSYDWWFRPKVFGGGTKLTVLGQPKAAPSVTLFPPSSEELQANKATLVCLISDFYPGAVTVAWKADSSPVKAGVETTTPSKQSNNKYAASSYLSLTPEQWKSHRSYSCQVTHEGSTVEKTVAPTECS

SEQ ID NO: 89 - DNA, 654 bp, Artificial Sequence
  anti-CD47 Kc4F4 kappa light chain
cagtctgccctgactcagcctgcctccgtgtctgggtctcctggacagtcgatcaccatctcctgcactggaaccagcagtgacgttaggagggctaactatgtctcctggtaccaacagcacccaggcaaagcccccaaactcatgatttatcaggatagtagtcggccctcaggggtttctaatcgcttctctggctccaagtctggcaacacggcctccctgaccatctctgggctccaggctgaggacgaggctgattattactgcagctcatatgattggtggttccgccccaaggtgttcggcggagggaccaagctgaccgtcctaggtcagcccaaggctgccccctcggtcactctgttcccgccctcctctgaggagcttcaagccaacaaggccacactggtgtgtctcataagtgacttctacccgggagccgtgacagtggcttggaaagcagatagcagccccgtcaaggcgggagtggagaccaccacaccctccaaacaaagcaacaacaagtacgcggccagcagctatctgagcctgacgcctgagcagtggaagtcccacagaagctacagctgccaggtcacgcatgaagggagcaccgtggagaagacagtggcccctacagaatgttcataa

SEQ ID NO: 90 - protein, 217 aa, Artificial Sequence
  anti-CD47 Kc4F4 kappa light chain
QSALTQPASVSGSPGQSITISCTGTSSDVRRANYVSWYQQHPGKAPKLMIYQDSSRPSGVSNRFSGSKSGNTASLTISGLQAEDEADYYCSSYDWWFRPKVFGGGTKLTVLGQPKAAPSVTLFPPSSEELQANKATLVCLISDFYPGAVTVAWKADSSPVKAGVETTTPSKQSNNKYAASSYLSLTPEQWKSHRSYSCQVTHEGSTVEKTVAPTECS

SEQ ID NO: 91 - DNA, 654 bp, Artificial Sequence
  anti-CD47 Kc4B1 kappa light chain
cagtctgccctgactcagcctgcctccgtgtctgggtctcctggacagtcgatcaccatctcctgcactggaaccagcagtgacgttagggctaataactatgtctcctggtaccaacagcacccaggcaaagcccccaaactcatgatttatgagagtagtgcgcggccctcaggggtttctaatcgcttctctggctccaagtctggcaacacggcctccctgaccatctctgggctccaggctgaggacgaggctgattattactgcagctcatatgattggtggttccgccccaaggtgttcggcggagggaccaagctgaccgtcctaggtcagcccaaggctgccccctcggtcactctgttcccgccctcctctgaggagcttcaagccaacaaggccacactggtgtgtctcataagtgacttctacccgggagccgtgacagtggcttggaaagcagatagcagccccgtcaaggcgggagtggagaccaccacaccctccaaacaaagcaacaacaagtacgcggccagcagctatctgagcctgacgcctgagcagtggaagtcccacagaagctacagctgccaggtcacgcatgaagggagcaccgtggagaagacagtggcccctacagaatgttcataa

SEQ ID NO: 92 - protein, 217 aa, Artificial Sequence
  anti-CD47 Kc4B1 kappa light chain
QSALTQPASVSGSPGQSITISCTGTSSDVRANNYVSWYQQHPGKAPKLMIYESSARPSGVSNRFSGSKSGNTASLTISGLQAEDEADYYCSSYDWWFRPKVFGGGTKLTVLGQPKAAPSVTLFPPSSEELQANKATLVCLISDFYPGAVTVAWKADSSPVKAGVETTTPSKQSNNKYAASSYLSLTPEQWKSHRSYSCQVTHEGSTVEKTVAPTECS

SEQ ID NO: 93 - DNA, 654 bp, Artificial Sequence
  anti-CD47 Kc4E2 kappa light chain
cagtctgccctgactcagcctgcctccgtgtctgggtctcctggacagtcgatcaccatctcctgcactggaaccagcagtgacgtttattataataagtatgtctcctggtaccaacagcacccaggcaaagcccccaaactcatgatttatgagagtagtaagcggccctcaggggtttctaatcgcttctctggctccaagtctggcaacacggcctccctgaccatctctgggctccaggctgaggacgaggctgattattactgcagctcatatgattggtggttccgccccaaggtgttcggcggagggaccaagctgaccgtcctaggtcagcccaaggctgccccctcggtcactctgttcccgccctcctctgaggagcttcaagccaacaaggccacactggtgtgtctcataagtgacttctacccgggagccgtgacagtggcttggaaagcagatagcagccccgtcaaggcgggagtggagaccaccacaccctccaaacaaagcaacaacaagtacgcggccagcagctatctgagcctgacgcctgagcagtggaagtcccacagaagctacagctgccaggtcacgcatgaagggagcaccgtggagaagacagtggcccctacagaatgttcataa

SEQ ID NO: 94 - protein, 217 aa, Artificial Sequence
  anti-CD47 Kc4E2 kappa light chain
QSALTQPASVSGSPGQSITISCTGTSSDVYYNKYVSWYQQHPGKAPKLMIYESSKRPSGVSNRFSGSKSGNTASLTISGLQAEDEADYYCSSYDWWFRPKVFGGGTKLTVLGQPKAAPSVTLFPPSSEELQANKATLVCLISDFYPGAVTVAWKADSSPVKAGVETTTPSKQSNNKYAASSYLSLTPEQWKSHRSYSCQVTHEGSTVEKTVAPTECS

SEQ ID NO: 95 - DNA, 657 bp, Artificial Sequence
  anti-CD19 C2 lambda light chain
aattttatgctgactcagccccactctgtgtcggagtctccggggaagacggtaaccatctcctgcacccgcagcagtggctctatcgaagataagtatgtgcagtggtaccagcagcgcccgggcagttcccccaccattgtgatctattatgataacgaaagaccctctggggtccctgatcggttctctggctccatcgacagctcctccaactctgcctccctcaccatctctggactgaagactgaggacgaggctgactactactgtcagacctacgaccagagcctgtatggttgggtgttcggcggagggaccaagctgaccgtcctaggtcagcccaaggctgccccctcggtcactctgttcccgccctcctctgaggagcttcaagccaacaaggccacactggtgtgtctcataagtgacttctacccgggagccgtgacagtggcttggaaagcagatagcagccccgtcaaggcgggagtggagaccaccacaccctccaaacaaagcaacaacaagtacgcggccagcagctatctgagcctgacgcctgagcagtggaagtcccacagaagctacagctgccaggtcacgcatgaagggagcaccgtggagaagacagtggcccctacagaatgttcataa

SEQ ID NO: 96 - protein, 218 aa, Artificial Sequence
  anti-CD19 C2 lambda light chain
NFMLTQPHSVSESPGKTVTISCTRSSGSIEDKYVQWYQQRPGSSPTIVIYYDNERPSGVPDRFSGSIDSSSNSASLTISGLKTEDEADYYCQTYDQSLYGWVFGGGTKLTVLGQPKAAPSVTLFPPSSEELQANKATLVCLISDFYPGAVTVAWKADSSPVKAGVETTTPSKQSNNKYAASSYLSLTPEQWKSHRSYSCQVTHEGSTVEKTVAPTECS

SEQ ID NO: 97 - DNA, 657 bp, Artificial Sequence
  anti-CD19 A6 lambda light chain
aattttatgctgactcagccccactctgtgtcggagtctccggggaagacggtaaccatctcctgcacccgcagcagtggctctatcggtgataagtatgtgcagtggtaccagcagcgcccgggcagttcccccaccattgtgatctattatgataacgaaagaccctctggggtccctgatcggttctctggctccatcgacagctcctccaactctgcctccctcaccatctctggactgaagactgaggacgaggctgactactactgtcagacgtacgacgagagcctgtatggttgggtgttcggcggagggaccaagctgaccgtcctaggtcagcccaaggctgccccctcggtcactctgttcccgccctcctctgaggagcttcaagccaacaaggccacactggtgtgtctcataagtgacttctacccgggagccgtgacagtggcttggaaagcagatagcagccccgtcaaggcgggagtggagaccaccacaccctccaaacaaagcaacaacaagtacgcggccagcagctatctgagcctgacgcctgagcagtggaagtcccacagaagctacagctgccaggtcacgcatgaagggagcaccgtggagaagacagtggcccctacagaatgttcataa

SEQ ID NO: 98 - protein, 218 aa, Artificial Sequence
  anti-CD19 A6 lambda light chain
NFMLTQPHSVSESPGKTVTISCTRSSGSIGDKYVQWYQQRPGSSPTIVIYYDNERPSGVPDRFSGSIDSSSNSASLTISGLKTEDEADYYCQTYDESLYGWVFGGGTKLTVLGQPKAAPSVTLFPPSSEELQANKATLVCLISDFYPGAVTVAWKADSSPVKAGVETTTPSKQSNNKYAASSYLSLTPEQWKSHRSYSCQVTHEGSTVEKTVAPTECS

SEQ ID NO: 99 - DNA, 657 bp, Artificial Sequence
  anti-CD19 C6 lambda light chain
aattttatgctgactcagccccactctgtgtcggagtctccggggaagacggtaaccatctcctgcacccgcagcagtggctctatcaatgataagtatgtgcagtggtaccagcagcgcccgggcagttcccccaccattgtgatctattttgataacgaaagaccctctggggtccctgatcggttctctggctccatcgacagctcctccaactctgcctccctcaccatctctggactgaagactgaggacgaggctgactactactgtcagacctacgacaccagcctgtatggttgggtgttcggcggagggaccaagctgaccgtcctaggtcagcccaaggctgccccctcggtcactctgttcccgccctcctctgaggagcttcaagccaacaaggccacactggtgtgtctcataagtgacttctacccgggagccgtgacagtggcttggaaagcagatagcagccccgtcaaggcgggagtggagaccaccacaccctccaaacaaagcaacaacaagtacgcggccagcagctatctgagcctgacgcctgagcagtggaagtcccacagaagctacagctgccaggtcacgcatgaagggagcaccgtggagaagacagtggcccctacagaatgttcataa

SEQ ID NO: 100 - protein, 218 aa, Artificial Sequence
  anti-CD19 C6 lambda light chain
NFMLTQPHSVSESPGKTVTISCTRSSGSINDKYVQWYQQRPGSSPTIVIYFDNERPSGVPDRFSGSIDSSSNSASLTISGLKTEDEADYYCQTYDTSLYGWVFGGGTKLTVLGQPKAAPSVTLFPPSSEELQANKATLVCLISDFYPGAVTVAWKADSSPVKAGVETTTPSKQSNNKYAASSYLSLTPEQWKSHRSYSCQVTHEGSTVEKTVAPTECS

SEQ ID NO: 101 - DNA, 657 bp, Artificial Sequence
  anti-CD19 C9 lambda light chain
aattttatgctgactcagccccactctgtgtcggagtctccggggaagacggtaaccatctcctgcacccgcagcagtggctctatcgctgataagtatgtgcagtggtaccagcagcgcccgggcagttcccccaccattgtgatctattatgataacgaaagaccctctggggtccctgatcggttctctggctccatcgacagctcctccaactctgcctccctcaccatctctggactgaagactgaggacgaggctgactactactgtcagacctacgacgagagcctgtatggttgggtgttcggcggagggaccaagctgaccgtcctaggtcagcccaaggctgccccctcggtcactctgttcccgccctcctctgaggagcttcaagccaacaaggccacactggtgtgtctcataagtgacttctacccgggagccgtgacagtggcttggaaagcagatagcagccccgtcaaggcgggagtggagaccaccacaccctccaaacaaagcaacaacaagtacgcggccagcagctatctgagcctgacgcctgagcagtggaagtcccacagaagctacagctgccaggtcacgcatgaagggagcaccgtggagaagacagtggcccctacagaatgttcataa

SEQ ID NO: 102 - protein, 218 aa, Artificial Sequence
  anti-CD19 C9 lambda light chain
NFMLTQPHSVSESPGKTVTISCTRSSGSIADKYVQWYQQRPGSSPTIVIYYDNERPSGVPDRFSGSIDSSSNSASLTISGLKTEDEADYYCQTYDESLYGWVFGGGTKLTVLGQPKAAPSVTLFPPSSEELQANKATLVCLISDFYPGAVTVAWKADSSPVKAGVETTTPSKQSNNKYAASSYLSLTPEQWKSHRSYSCQVTHEGSTVEKTVAPTECS

SEQ ID NO: 103 - DNA, 657 bp, Artificial Sequence
  anti-CD19 B11 lambda light chain
aattttatgctgactcagccccactctgtgtcggagtctccggggaagacggtaaccatctcctgcacccgcagcagtggctctatcgaagataagtatgtgcagtggtaccagcagcgcccgggcagttcccccaccattgtgatctattatgataacgaaagaccctctggggtccctgatcggttctctggctccatcgacagctcctccaactctgcctccctcaccatctctggactgaagactgaggacgaggctgactactactgtcagacctacgacaacagcctgtatggttgggtgttcggcggagggaccaagctgaccgtcctaggtcagcccaaggctgccccctcggtcactctgttcccgccctcctctgaggagcttcaagccaacaaggccacactggtgtgtctcataagtgacttctacccgggagccgtgacagtggcttggaaagcagatagcagccccgtcaaggcgggagtggagaccaccacaccctccaaacaaagcaacaacaagtacgcggccagcagctatctgagcctgacgcctgagcagtggaagtcccacagaagctacagctgccaggtcacgcatgaagggagcaccgtggagaagacagtggcccctacagaatgttcataa

SEQ ID NO: 104 - protein, 218 aa, Artificial Sequence
  anti-CD19 B11 lambda light chain
NFMLTQPHSVSESPGKTVTISCTRSSGSIEDKYVQWYQQRPGSSPTIVIYYDNERPSGVPDRFSGSIDSSSNSASLTISGLKTEDEADYYCQTYDNSLYGWVFGGGTKLTVLGQPKAAPSVTLFPPSSEELQANKATLVCLISDFYPGAVTVAWKADSSPVKAGVETTTPSKQSNNKYAASSYLSLTPEQWKSHRSYSCQVTHEGSTVEKTVAPTECS

SEQ ID NO: 105 - DNA, 657 bp, Artificial Sequence
  anti-CD19 D11 lambda light chain
aattttatgctgactcagccccactctgtgtcggagtctccggggaagacggtaaccatctcctgcacccgcagcagtggcagcatcgatgataagtttgtgcagtggtaccagcagcgcccgggcagttcccccaccactgtgatctattatgataacattagaccctctggggtccctgatcggttctctggctccatcgacagctcctccaactctgcctccctcaccatctctggactgaagactgaggacgaggctgactactactgtcagtcctatgacgcgagcctgtatggttgggtgttcggcggagggaccaagctgaccgtcctaggtcagcccaaggctgccccctcggtcactctgttcccgccctcctctgaggagcttcaagccaacaaggccacactggtgtgtctcataagtgacttctacccgggagccgtgacagtggcttggaaagcagatagcagccccgtcaaggcgggagtggagaccaccacaccctccaaacaaagcaacaacaagtacgcggccagcagctatctgagcctgacgcctgagcagtggaagtcccacagaagctacagctgccaggtcacgcatgaagggagcaccgtggagaagacagtggcccctacagaatgttcataa

SEQ ID NO: 106 - protein, 218 aa, Artificial Sequence
  anti-CD19 D11 lambda light chain
NFMLTQPHSVSESPGKTVTISCTRSSGSIDDKFVQWYQQRPGSSPTTVIYYDNIRPSGVPDRFSGSIDSSSNSASLTISGLKTEDEADYYCQSYDASLYGWVFGGGTKLTVLGQPKAAPSVTLFPPSSEELQANKATLVCLISDFYPGAVTVAWKADSSPVKAGVETTTPSKQSNNKYAASSYLSLTPEQWKSHRSYSCQVTHEGSTVEKTVAPTECS

SEQ ID NO: 107 - DNA, 657 bp, Artificial Sequence
  anti-CD19 B7 lambda light chain
aattttatgctgactcagccccactctgtgtcggagtctccggggaagacggtaaccatctcctgcacccgcagcagtggctctatcgcggataagtatgtgcagtggtaccagcagcgcccgggcagttcccccaccactgtgatctatgaggataaccaaagaccctctggggtccctgatcggttctctggctccatcgacagctcctccaactctgcctccctcaccatctctggactgaagactgaggacgaggctgactactactgtcagtcctatgacagcagcctgtatggttgggtgttcggcggagggaccaagctgaccgtcctaggtcagcccaaggctgccccctcggtcactctgttcccgccctcctctgaggagcttcaagccaacaaggccacactggtgtgtctcataagtgacttctacccgggagccgtgacagtggcttggaaagcagatagcagccccgtcaaggcgggagtggagaccaccacaccctccaaacaaagcaacaacaagtacgcggccagcagctatctgagcctgacgcctgagcagtggaagtcccacagaagctacagctgccaggtcacgcatgaagggagcaccgtggagaagacagtggcccctacagaatgttcataa

SEQ ID NO: 108 - protein, 218 aa, Artificial Sequence
  anti-CD19 B7 lambda light chain
NFMLTQPHSVSESPGKTVTISCTRSSGSIADKYVQWYQQRPGSSPTTVIYEDNQRPSGVPDRFSGSIDSSSNSASLTISGLKTEDEADYYCQSYDSSLYGWVFGGGTKLTVLGQPKAAPSVTLFPPSSEELQANKATLVCLISDFYPGAVTVAWKADSSPVKAGVETTTPSKQSNNKYAASSYLSLTPEQWKSHRSYSCQVTHEGSTVEKTVAPTECS

SEQ ID NO: 109 - DNA, 651 bp, Artificial Sequence
  dummy light chain 1
cagtctgtgttgacgcagccgccctcagtgtctgcggccccaggacagaaggtcaccatctcctgctctggaagcagctccaatattgagactggttctgtatcctggtaccagcagctcccaggaacagcccccaaactcctcatttatgacaataataagcgaccctcagggattcctgaccgattctctggctccaagtctggcacgtcagccaccctgggcatcaccggactccagactggggacgaggccgattattactgcggaacatgggatgacagcctgcctggatgggtgttcggcggagggaccaagctgaccgtcctaggtcagcccaaggctgccccctcggtcactctgttcccgccctcctctgaggagcttcaagccaacaaggccacactggtgtgtctcataagtgacttctacccgggagccgtgacagtggcttggaaagcagatagcagccccgtcaaggcgggagtggagaccaccacaccctccaaacaaagcaacaacaagtacgcggccagcagctatctgagcctgacgcctgagcagtggaagtcccacagaagctacagctgccaggtcacgcatgaagggagcaccgtggagaagacagtggcccctacagaatgttcataa

SEQ ID NO: 110 - protein, 216 aa, Artificial Sequence
  dummy light chain 1
QSVLTQPPSVSAAPGQKVTISCSGSSSNIETGSVSWYQQLPGTAPKLLIYDNNKRPSGIPDRFSGSKSGTSATLGITGLQTGDEADYYCGTWDDSLPGWVFGGGTKLTVLGQPKAAPSVTLFPPSSEELQANKATLVCLISDFYPGAVTVAWKADSSPVKAGVETTTPSKQSNNKYAASSYLSLTPEQWKSHRSYSCQVTHEGSTVEKTVAPTECS

SEQ ID NO: 111 - DNA, 657 bp, Artificial Sequence
  dummy light chain 2
gaaatagtgatgacgcagtctccagccaccctgtctgtgtctccaggggaaagagccaccctctcctgcagggccagtcagacggttaagaataatttagcctggtaccagcagaaacctggccaggctcccaggctcctcatctatggtgcatccaccagggccactggtatcccagccaggttcagtggcagtgggtctgggacagagttcactctcaccatcagcagcctgcagtctgaagattttgcagtttattactgtcagcagtataacaactggttgcccatcaacccctataccttcggccaagggaccaaggtggaaatcaaacgtacggtggctgcaccatctgtcttcatcttcccgccatctgatgagcagttgaaatctggaactgcctctgttgtgtgcctgctgaataacttctatcccagagaggccaaagtacagtggaaggtggataacgccctccaatcgggtaactcccaggagagtgtcacagagcaggacagcaaggacagcacctacagcctcagcagcaccctgacgctgagcaaagcagactacgagaaacacaaagtctacgcctgcgaagtcacccatcagggcctgagctcgcccgtcacaaagagcttcaacaggggagagtgttaa

SEQ ID NO: 112 - protein, 218 aa, Artificial Sequence
  dummy light chain 2
EIVMTQSPATLSVSPGERATLSCRASQTVKNNLAWYQQKPGQAPRLLIYGASTRATGIPARFSGSGSGTEFTLTISSLQSEDFAVYYCQQYNNWLPINPYTFGQGTKVEIKRTVAAPSVFIFPPSDEQLKSGTASVVCLLNNFYPREAKVQWKVDNALQSGNSQESVTEQDSKDSTYSLSSTLTLSKADYEKHKVYACEVTHQGLSSPVTKSFNRGEC

SEQ ID NO: 113 - DNA, 348 bp, Artificial Sequence
  common variable heavy domain
gaggtgcagctgttggagtctgggggaggcttggtacagcctggggggtccctgagactctcctgtgcagcctctggattcacctttagcagctatgccatgagctgggtccgccaggctccagggaaggggctggagtgggtctcagctattagtggtagtggtggtagcacatactacgcagactccgtgaagggccggttcaccatctccagagacaattccaagaacacgctgtatctgcaaatgaacagcctgagagccgaggacacggccgtatattactgtgcgaaaagttatggtgcttttgactactggggccagggaaccctggtcacagtctcgagc

SEQ ID NO: 114 - protein, 116 aa, Artificial Sequence
  common variable heavy domain
EVQLLESGGGLVQPGGSLRLSCAASGFTFSSYAMSWVRQAPGKGLEWVSAISGSGGSTYYADSVKGRFTISRDNSKNTLYLQMNSLRAEDTAVYYCAKSYGAFDYWGQGTLVTVSS

SEQ ID NO: 115 - DNA, 324 bp, Artificial Sequence
  anti-CD47 5A3 kappa variable light domain
gacatccagatgacccagtctccatcctccctgtctgcatctgtaggagacagagtcaccatcacttgccaggcgagtcaggacattaataagtatttaaattggtatcagcagaaaccagggaaagcccctaagctcctgatctacggtgcatccaggttggaaacaggggtcccatcaaggttcagtggaagtggatctgggacagattttactttcaccatcagcagcctgcagcctgaagatattgcaacatattactgtcagcagaagcacccccgggggccgaggaccttcggccaagggaccaaggtggaaatcaaa

SEQ ID NO: 116 - protein, 108 aa, Artificial Sequence
  anti-CD47 5A3 kappa variable light domain
DIQMTQSPSSLSASVGDRVTITCQASQDINKYLNWYQQKPGKAPKLLIYGASRLETGVPSRFSGSGSGTDFTFTISSLQPEDIATYYCQQKHPRGPRTFGQGTKVEIK

SEQ ID NO: 117 - DNA, 324 bp, Artificial Sequence
  anti-CD47 5A3-M4  kappa variable light domain
gacatccagatgacccagtctccatcctccctgtctgcatctgtaggagacagagtcaccatcacttgccaggcgagtcaggacattaataagtatttaaattggtatcagcagaaaccagggaaagcccctaagctcctgatctacggtgcatccaggttggaaacaggggtcccatcaaggttcagtggaagtggatctgggacagattttactttcaccatcagcagcctgcagcctgaagatattgcaacatattactgtcagcagaagcacccccggaacccgaggaccttcggccaagggaccaaggtggaaatcaaa

SEQ ID NO: 118 - protein, 108 aa, Artificial Sequence
  anti-CD47 5A3-M4  kappa variable light domain
DIQMTQSPSSLSASVGDRVTITCQASQDINKYLNWYQQKPGKAPKLLIYGASRLETGVPSRFSGSGSGTDFTFTISSLQPEDIATYYCQQKHPRNPRTFGQGTKVEIK

SEQ ID NO: 119 - DNA, 324 bp, Artificial Sequence
  anti-CD47 5A3-M3  kappa variable light domain
gacatccagatgacccagtctccatcctccctgtctgcatctgtaggagacagagtcaccatcacttgccaggcgagtcagtccattagtagttatttaaattggtatcagcagaaaccagggaaagcccctaagctcctgatctacgctgcatcctcgttggaaacaggggtcccatcaaggttcagtggaagtggatctgggacagattttactttcaccatcagcagcctgcagcctgaagatattgcaacatattactgtcagcagaagcacccccgggggccgaggaccttcggccaagggaccaaggtggaaatcaaa

SEQ ID NO: 120 - protein, 108 aa, Artificial Sequence
  anti-CD47 5A3-M3  kappa variable light domain
DIQMTQSPSSLSASVGDRVTITCQASQSISSYLNWYQQKPGKAPKLLIYAASSLETGVPSRFSGSGSGTDFTFTISSLQPEDIATYYCQQKHPRGPRTFGQGTKVEIK

SEQ ID NO: 121 - DNA, 324 bp, Artificial Sequence
  anti-CD47 5A3-M5 kappa variable light domain
gacatccagatgacccagtctccatcctccctgtctgcatctgtaggagacagagtcaccatcacttgccaggcgagtcaggacattaataagtatttaaattggtatcagcagaaaccagggaaagcccctaagctcctgatctacggtgcatccaggttggaaacaggggtcccatcaaggttcagtggaagtggatctgggacagattttactttcaccatcagcagcctgcagcctgaagatattgcaacatattactgtcagcagaagcacccccggtacccgaggaccttcggccaagggaccaaggtggaaatcaaa

SEQ ID NO: 122 - protein, 108 aa, Artificial Sequence
  anti-CD47 5A3-M5 kappa variable light domain
DIQMTQSPSSLSASVGDRVTITCQASQDINKYLNWYQQKPGKAPKLLIYGASRLETGVPSRFSGSGSGTDFTFTISSLQPEDIATYYCQQKHPRYPRTFGQGTKVEIK

SEQ ID NO: 123 - DNA, 324 bp, Artificial Sequence
  anti-CD47 Ke8 kappa variable light domain
gacatccagatgacccagtctccatcctccctgtctgcatctgtaggagacagagtcaccatcacttgccgggcaagtcagagcattagcagctatttaaattggtatcagcagaaaccagggaaagcccctaagctcctgatctatgctgcatccagtttgcaaagtggggtcccatcaaggttcagtggcagtggatctgggacagatttcactctcaccatcagcagtctgcaacctgaagattttgcaacttactactgtcagcagttccacaagcggcggccgcagaccttcggccaagggaccaaggtggaaatcaaa

SEQ ID NO: 124 - protein, 108 aa, Artificial Sequence
  anti-CD47 Ke8 kappa variable light domain
DIQMTQSPSSLSASVGDRVTITCRASQSISSYLNWYQQKPGKAPKLLIYAASSLQSGVPSRFSGSGSGTDFTLTISSLQPEDFATYYCQQFHKRRPQTFGQGTKVEIK

SEQ ID NO: 125 - DNA, 324 bp, Artificial Sequence
  anti-CD47 Ke8H5 kappa variable light domain
gacatccagatgacccagtctccatcctccctgtctgcatctgtaggagacagagtcaccatcacttgccgggcaagtcagagcattgcgaggtatttaaattggtatcagcagaaaccagggaaagcccctaagctcctgatctatgctgcatccagtttgcaaagtggggtcccatcaaggttcagtggcagtggatctgggacagatttcactctcaccatcagcagtctgcaacctgaagattttgcaacttactactgtcagcagttccataagcgtgcgccgcagaccttcggccaagggaccaaggtggaaatcaaa

SEQ ID NO: 126 - protein, 108 aa, Artificial Sequence
  anti-CD47 Ke8H5 kappa variable light domain
DIQMTQSPSSLSASVGDRVTITCRASQSIARYLNWYQQKPGKAPKLLIYAASSLQSGVPSRFSGSGSGTDFTLTISSLQPEDFATYYCQQFHKRAPQTFGQGTKVEIK

SEQ ID NO: 127 - DNA, 324 bp, Artificial Sequence
  anti-CD47 Ke8B2 kappa variable light domain
gacatccagatgacccagtctccatcctccctgtctgcatctgtaggagacagagtcaccatcacttgccgggcaagtcagagcattggtaagtatttaaattggtatcagcagaaaccagggaaagcccctaagctcctgatctatgcggcatccaggttgcaaagtggggtcccatcaaggttcagtggcagtggatctgggacagatttcactctcaccatcagcagtctgcaacctgaagattttgcaacttactactgtcagcagaagcacccgcgtgccccgcggaccttcggccaagggaccaaggtggaaatcaaa

SEQ ID NO: 128 - protein, 108 aa, Artificial Sequence
  anti-CD47 Ke8B2 kappa variable light domain
DIQMTQSPSSLSASVGDRVTITCRASQSIGKYLNWYQQKPGKAPKLLIYAASRLQSGVPSRFSGSGSGTDFTLTISSLQPEDFATYYCQQKHPRAPRTFGQGTKVEIK

SEQ ID NO: 129 - DNA, 324 bp, Artificial Sequence
  anti-CD47 Ke8A2 kappa variable light domain
gacatccagatgacccagtctccatcctccctgtctgcatctgtaggagacagagtcaccatcacttgccgggcaagtcagagcattgataggtatttaaattggtatcagcagaaaccagggaaagcccctaagctcctgatctatgctgcatccagtttgcaaagtggggtcccatcaaggttcagtggcagtggatctgggacagatttcactctcaccatcagcagtctgcaacctgaagattttgcaacttactactgtcagcagaagcatccccgtgggccgaggaccttcggccaagggaccaaggtggaaatcaaa

SEQ ID NO: 130 - protein, 108 aa, Artificial Sequence
  anti-CD47 Ke8A2 kappa variable light domain
DIQMTQSPSSLSASVGDRVTITCRASQSIDRYLNWYQQKPGKAPKLLIYAASSLQSGVPSRFSGSGSGTDFTLTISSLQPEDFATYYCQQKHPRGPRTFGQGTKVEIK

SEQ ID NO: 131 - DNA, 324 bp, Artificial Sequence
  anti-CD47 Ke8E8 kappa variable light domain
gacatccagatgacccagtctccatcctccctgtctgcatctgtaggagacagagtcaccatcacttgccaggcgagtcaggacattaataagtatttaaattggtatcagcagaaaccagggaaagcccctaagctcctgatctatgctgcatccagtttgcaaagtggggtcccatcaaggttcagtggcagtggatctgggacagatttcactctcaccatcagcagtctgcaacctgaagattttgcaacttactactgtcagcagaagcatccccgtggcccgcggaccttcggccaagggaccaaggtggaaatcaaa

SEQ ID NO: 132 - protein, 108 aa, Artificial Sequence
  anti-CD47 Ke8E8 kappa variable light domain
DIQMTQSPSSLSASVGDRVTITCQASQDINKYLNWYQQKPGKAPKLLIYAASSLQSGVPSRFSGSGSGTDFTLTISSLQPEDFATYYCQQKHPRGPRTFGQGTKVEIK

SEQ ID NO: 133 - DNA, 324 bp, Artificial Sequence
  anti-CD47 Ke8H3 kappa variable light domain
gacatccagatgacccagtctccatcctccctgtctgcatctgtaggagacagagtcaccatcacttgccgggcaagtcagagcattaataggtatttaaattggtatcagcagaaaccagggaaagcccctaagctcctgatctatgctgcatccaggttgcaaagtggggtcccatcaaggttcagtggcagtggatctgggacagatttcactctcaccatcagcagtctgcaacctgaagattttgcaacttactactgtcagcagaagcatccgcgtgggccgaggaccttcggccaagggaccaaggtggaaatcaaa

SEQ ID NO: 134 - protein, 108 aa, Artificial Sequence
  anti-CD47 Ke8H3 kappa variable light domain
DIQMTQSPSSLSASVGDRVTITCRASQSINRYLNWYQQKPGKAPKLLIYAASRLQSGVPSRFSGSGSGTDFTLTISSLQPEDFATYYCQQKHPRGPRTFGQGTKVEIK

SEQ ID NO: 135 - DNA, 324 bp, Artificial Sequence
  anti-CD47 Ke8G6 kappa variable light domain
gacatccagatgacccagtctccatcctccctgtctgcatctgtaggagacagagtcaccatcacttgccgggcaagtcagagcattggtaggtatttaaattggtatcagcagaaaccagggaaagcccctaagctcctgatctatgctgcatccagtttgcaaagtggggtcccatcaaggttcagtggcagtggatctgggacagatttcactctcaccatcagcagtctgcaacctgaagattttgcaacttactactgtcagcagatgcatccgcgtgcgccgaagaccttcggccaagggaccaaggtggaaatcaaa

SEQ ID NO: 136 - protein, 108 aa, Artificial Sequence
  anti-CD47 Ke8G6 kappa variable light domain
DIQMTQSPSSLSASVGDRVTITCRASQSIGRYLNWYQQKPGKAPKLLIYAASSLQSGVPSRFSGSGSGTDFTLTISSLQPEDFATYYCQQMHPRAPKTFGQGTKVEIK

SEQ ID NO: 137 - DNA, 324 bp, Artificial Sequence
  anti-CD47 Ke8A3 kappa variable light domain
gacatccagatgacccagtctccatcctccctgtctgcatctgtaggagacagagtcaccatcacttgccgggtaagtcagagcattagtaagtatttaaattggtatcagcagaaaccagggaaagcccctaagctcctgatctatgctgcatccagtttgcaaagtggggtcccatcaaggttcagtggcagtggatctgggacagatttcactctcaccatcagcagtctgcaacctgaagattttgcaacttactactgtcagcagaggcatccccgtgggccgagcaccttcggccaagggaccaaggtggaaatcaaa

SEQ ID NO: 138 - protein, 108 aa, Artificial Sequence
  anti-CD47 Ke8A3 kappa variable light domain
DIQMTQSPSSLSASVGDRVTITCRVSQSISKYLNWYQQKPGKAPKLLIYAASSLQSGVPSRFSGSGSGTDFTLTISSLQPEDFATYYCQQRHPRGPSTFGQGTKVEIK

SEQ ID NO: 139 - DNA, 324 bp, Artificial Sequence
  anti-CD47 Ke81A3 kappa variable light domain
gacatccagatgacccagtctccatcctccctgtctgcatctgtaggagacagagtcaccatcacttgccaggcgagtcaggacattaataggtatttaaattggtatcagcagaaaccagggaaagcccctaagctcctgatctatgctgcatccagtttgcaaagtggggtcccatcaaggttcagtggcagtggatctgggacagatttcactctcaccatcagcagtctgcaacctgaagattttgcaacttactactgtcagcagaggcatccgcgtgccccgcggaccttcggccaagggaccaaggtggaaatcaaa

SEQ ID NO: 140 - protein, 108 aa, Artificial Sequence
  anti-CD47 Ke81A3 kappa variable light domain
DIQMTQSPSSLSASVGDRVTITCQASQDINRYLNWYQQKPGKAPKLLIYAASSLQSGVPSRFSGSGSGTDFTLTISSLQPEDFATYYCQQRHPRAPRTFGQGTKVEIK

SEQ ID NO: 141 - DNA, 324 bp, Artificial Sequence
  anti-CD47 Ke8A8 kappa variable light domain
gacatccagatgacccagtctccatcctccctgtctgcatctgtaggagacagagtcaccatcacttgccgggcaagtcagagcattagtaagtatttaaattggtatcagcagaaaccagggaaagcccctaagctcctgatctatgctgcatccactttgcaaagtggggtcccatcaaggttcagtggcagtggatctgggacagatttcactctcaccatcagcagtctgcaacctgaagattttgcaacttactactgtcagcagatgcatccgcgtgcgccgaagaccttcggccaagggaccaaggtggaaatcaaa

SEQ ID NO: 142 - protein, 108 aa, Artificial Sequence
  anti-CD47 Ke8A8 kappa variable light domain
DIQMTQSPSSLSASVGDRVTITCRASQSISKYLNWYQQKPGKAPKLLIYAASTLQSGVPSRFSGSGSGTDFTLTISSLQPEDFATYYCQQMHPRAPKTFGQGTKVEIK

SEQ ID NO: 143 - DNA, 324 bp, Artificial Sequence
  anti-CD47 Ke8C7 kappa variable light domain
gacatccagatgacccagtctccatcctccctgtctgcatctgtaggagacagagtcaccatcacttgccaggcgagtcaggacattaataggtatttaaattggtatcagcagaaaccagggaaagcccctaagctcctgatctatgctgcatccagtttgcaaagtggggtcccatcaaggttcagtggcagtggatctgggacagatttcactctcaccatcagcagtctgcaacctgaagattttgcaacttactactgtcagcagcgccatccgcgtggcccgaggaccttcggccaagggaccaaggtggaaatcaaa

SEQ ID NO: 144 - protein, 108 aa, Artificial Sequence
  anti-CD47 Ke8C7 kappa variable light domain
DIQMTQSPSSLSASVGDRVTITCQASQDINRYLNWYQQKPGKAPKLLIYAASSLQSGVPSRFSGSGSGTDFTLTISSLQPEDFATYYCQQRHPRGPRTFGQGTKVEIK

SEQ ID NO: 145 - DNA, 324 bp, Artificial Sequence
  anti-CD47 Ke8G2 kappa variable light domain
gacatccagatgacccagtctccatcctccctgtctgcatctgtaggagacagagtcaccatcacttgccgggcaagtcagagcattggtaggtatttaaattggtatcagcagaaaccagggaaagcccctaagctcctgatctatgcggcatccaggttgcaaagtggggtcccatcaaggttcagtggcagtggatctgggacagatttcactctcaccatcaacagtctgcaacctgaagattttgcaacttactactgtcagcagaagcatccccgtgcgccgaggaccttcggccaagggaccaaggtggaaatcaaa

SEQ ID NO: 146 - protein, 108 aa, Artificial Sequence
  anti-CD47 Ke8G2 kappa variable light domain
DIQMTQSPSSLSASVGDRVTITCRASQSIGRYLNWYQQKPGKAPKLLIYAASRLQSGVPSRFSGSGSGTDFTLTINSLQPEDFATYYCQQKHPRAPRTFGQGTKVEIK

SEQ ID NO: 147 - DNA, 324 bp, Artificial Sequence
  anti-CD47 Ke81G9 kappa variable light domain
gacatccagatgacccagtctccatcctccctgtctgcatctgtaggagacagagtcaccatcacttgccgggcaagtcagagcattgataagtatttaaattggtatcagcagaaaccagggaaagcccctaagctcctgatctatgcggcatccaggttgcaaagtggggtcccatcaaggttcagtggcagtggatctgggacagatttcactctcaccatcagcagtctgcaacctgaagattttgcaacttactactgtcagcagcggcataagcgttccccgcagaccttcggccaagggaccaaggtggaaatcaaa

SEQ ID NO: 148 - protein, 108 aa, Artificial Sequence
  anti-CD47 Ke81G9 kappa variable light domain
DIQMTQSPSSLSASVGDRVTITCRASQSIDKYLNWYQQKPGKAPKLLIYAASRLQSGVPSRFSGSGSGTDFTLTISSLQPEDFATYYCQQRHKRSPQTFGQGTKVEIK

SEQ ID NO: 149 - DNA, 324 bp, Artificial Sequence
  anti-CD47 Ke8F2 kappa variable light domain
gacatccagatgacccagtctccatcctccctgtctgcatctgtaggagacagagtcaccatcacttgccgggcaagtcagagcattgataagtatttaaattggtatcagcagaaaccagggaaagcccctaagctcctgatctatgctgcatccagtttgcaaagtggggtcccatcaaggttcagtggcagtggatctgggacagatttcactctcaccatcagcagtctgcaacctgaagattttgcaacttactactgtcagcagaagcatccgcgtgcgccgcggaccttcggccaagggaccaaggtggaaatcaaa

SEQ ID NO: 150 - protein, 108 aa, Artificial Sequence
  anti-CD47 Ke8F2 kappa variable light domain
DIQMTQSPSSLSASVGDRVTITCRASQSIDKYLNWYQQKPGKAPKLLIYAASSLQSGVPSRFSGSGSGTDFTLTISSLQPEDFATYYCQQKHPRAPRTFGQGTKVEIK

SEQ ID NO: 151 - DNA, 324 bp, Artificial Sequence
  anti-CD47 Ke8B7 kappa variable light domain
gacatccagatgacccagtctccatcctccctgtctgcatctgtaggagacagagtcaccatcacttgccgggcaagtcagagcattgggaagtatttaaattggtatcagcagaaaccagggaaagcccctaagctcctgatctatgctgcatccagtttgcaaagtggggtcccatcaaggttcagtggcagtggatctgggacagatttcactctcaccatcagcagtctgcaacctgaagattttgcaacttactactgtcagcagatgcatccgcgtagcccgaagaccttcggccaagggaccaaggtggaaatcaaa

SEQ ID NO: 152 - protein, 108 aa, Artificial Sequence
  anti-CD47 Ke8B7 kappa variable light domain
DIQMTQSPSSLSASVGDRVTITCRASQSIGKYLNWYQQKPGKAPKLLIYAASSLQSGVPSRFSGSGSGTDFTLTISSLQPEDFATYYCQQMHPRSPKTFGQGTKVEIK

SEQ ID NO: 153 - DNA, 324 bp, Artificial Sequence
  anti-CD47 Ke8C4 kappa variable light domain
gacatccagatgacccagtctccatcctccctgtctgcatctgtaggagacagagtcaccatcacttgccgggcaagtcagagcattagtaggtatttaaattggtatcagcagaaaccagggaaagcccctaagctcctgatctatgctgcatccaatttgcaaagtggggtcccatcaaggttcagtggcagtggatctgggacagatttcactctcaccatcagcagtctgcaacctgaagattttgcaacttactactgtcagcagatgcatccgcgtgggccgaagaccttcggccaagggaccaaggtggaaatcaaa

SEQ ID NO: 154 - protein, 108 aa, Artificial Sequence
  anti-CD47 Ke8C4 kappa variable light domain
DIQMTQSPSSLSASVGDRVTITCRASQSISRYLNWYQQKPGKAPKLLIYAASNLQSGVPSRFSGSGSGTDFTLTISSLQPEDFATYYCQQMHPRGPKTFGQGTKVEIK

SEQ ID NO: 155 - DNA, 324 bp, Artificial Sequence
  anti-CD47 Ke8F1 kappa variable light domain
gacatccagatgacccagtctccatcctccctgtctgcatctgtaggagacagagtcaccatcacttgccgggcaagtcagagcattgcttcttatgtaaattggtatcagcagaaaccagggaaagcccctaagctcctgatctatgctgcatccggtttgcaaagtggggtcccatcaaggttcagtggcagtggatctgggacagatttcactctcaccatcagcagtctgcaacctgaagattttgcaacttactactgtcagcagttccataagcgtcggccgcagaccttcggccaagggaccaaggtggaaatcaaa

SEQ ID NO: 156 - protein, 108 aa, Artificial Sequence
  anti-CD47 Ke8F1 kappa variable light domain
DIQMTQSPSSLSASVGDRVTITCRASQSIASYVNWYQQKPGKAPKLLIYAASGLQSGVPSRFSGSGSGTDFTLTISSLQPEDFATYYCQQFHKRRPQTFGQGTKVEIK

SEQ ID NO: 157 - DNA, 324 bp, Artificial Sequence
  anti-CD47 Ke8G11 kappa variable light domain
gacatccagatgacccagtctccatcctccctgtctgcatctgtaggagacagagtcaccatcacttgccgggcaagtcagagcattgggaggtatttaaattggtatcagcagaaaccagggaaagcccctaagctcctgatctatgctgcatccagtttgcaaagtggggtcccatcaaggttcagtggcagtggatctgggacagatttcactctcaccatcagcagtctgcaacctgaagattttgcaacttactactgtcagcagatgcatccgcgtgggccgaagaccttcggccaagggaccaaggtggaaatcaaa

SEQ ID NO: 158 - protein, 108 aa, Artificial Sequence
  anti-CD47 Ke8G11 kappa variable light domain
DIQMTQSPSSLSASVGDRVTITCRASQSIGRYLNWYQQKPGKAPKLLIYAASSLQSGVPSRFSGSGSGTDFTLTISSLQPEDFATYYCQQMHPRGPKTFGQGTKVEIK

SEQ ID NO: 159 - DNA, 324 bp, Artificial Sequence
  anti-CD47 Ke8H6 kappa variable light domain
gacatccagatgacccagtctccatcctccctgtctgcatctgtaggagacagagtcaccatcacttgccgggcaagtcagagcattagtaagtatttaaattggtatcagcagaaaccagggaaagcccctaagctcctgatctataatgcatccactttgcaaagtggggtcccatcaaggttcagtggcagtggatctgggacagatttcactctcaccatcagcagtctgcaacctgaagattttgcaacttactactgtcagcagaggcatccgcgtgggccgcgcaccttcggccaagggaccaaggtggaaatcaaa

SEQ ID NO: 160 - protein, 108 aa, Artificial Sequence
  anti-CD47 Ke8H6 kappa variable light domain
DIQMTQSPSSLSASVGDRVTITCRASQSISKYLNWYQQKPGKAPKLLIYNASTLQSGVPSRFSGSGSGTDFTLTISSLQPEDFATYYCQQRHPRGPRTFGQGTKVEIK

SEQ ID NO: 161 - DNA, 324 bp, Artificial Sequence
  anti-CD47 Ke84G9 kappa variable light domain
gacatccagatgacccagtctccatcctccctgtctgcatctgtaggagacagagtcaccatcacttgccgggcaagtcagagcattagtaagtatttaaattggtatcagcagaaaccagggaaagcccctaagctcctgatctatgctgcatccagtttgcaaagtggggtcccatcaaggttcagtggcagtggatctgggacagatttcactctcaccatcagcagtctgcaacctgaagattttgcaacttactactgtcagcagaagcatccgcgtagcccgcggaccttcggccaagggaccaaggtggaaatcaaa

SEQ ID NO: 162 - protein, 108 aa, Artificial Sequence
  anti-CD47 Ke84G9 kappa variable light domain
DIQMTQSPSSLSASVGDRVTITCRASQSISKYLNWYQQKPGKAPKLLIYAASSLQSGVPSRFSGSGSGTDFTLTISSLQPEDFATYYCQQKHPRSPRTFGQGTKVEIK

SEQ ID NO: 163 - DNA, 324 bp, Artificial Sequence
  anti-CD47 Ke8A4 kappa variable light domain
gacatccagatgacccagtctccatcctccctgtctgcatctgtaggagacagagtcaccatcacttgccgggcaagtcagagcattgctaagtatttaaattggtatcagcagaaaccagggaaagcccctaagctcctgatctatgctgcatccagtttgcaaagtggggtcccatcaaggttcagtggcagtggatctgggacagatttcactctcaccatcagcagtctgcaacctgaagattttgcaacttactactgtcagcagttccataagcgtagcccgcagaccttcggccaagggaccaaggtggaaatcaaa

SEQ ID NO: 164 - protein, 108 aa, Artificial Sequence
  anti-CD47 Ke8A4 kappa variable light domain
DIQMTQSPSSLSASVGDRVTITCRASQSIAKYLNWYQQKPGKAPKLLIYAASSLQSGVPSRFSGSGSGTDFTLTISSLQPEDFATYYCQQFHKRSPQTFGQGTKVEIK

SEQ ID NO: 165 - DNA, 324 bp, Artificial Sequence
  anti-CD47 Ke86G9 kappa variable light domain
gacatccagatgacccagtctccatcctccctgtctgcatctgtaggagacagagtcaccatcacttgccgggcaagtcagagcattagtaagtatttaaattggtatcagcagaaaccagggaaagcccctaagctcctgatctataatgcatccaatttgcaaagtggggtcccatcaaggttcagtggcagtggatctgggacagatttcactctcaccatcagcagtctgcaacctgaagattttgcaacttactactgtcagcagaggcatccgcgtgggccgaccaccttcggccaagggaccaaggtggaaatcaaa

SEQ ID NO: 166 - protein, 108 aa, Artificial Sequence
  anti-CD47 Ke86G9 kappa variable light domain
DIQMTQSPSSLSASVGDRVTITCRASQSISKYLNWYQQKPGKAPKLLIYNASNLQSGVPSRFSGSGSGTDFTLTISSLQPEDFATYYCQQRHPRGPTTFGQGTKVEIK

SEQ ID NO: 167 - DNA, 324 bp, Artificial Sequence
  anti-CD47 Ka3 kappa variable light domain
gacatccagatgacccagtctccatcctccctgtctgcatctgtaggagacagagtcaccatcacttgccgggcaagtcagagcattagcagctatttaaattggtatcagcagaaaccagggaaagcccctaagctcctgatctatgctgcatccagtttgcaaagtggggtcccatcaaggttcagtggcagtggatctgggacagatttcactctcaccatcagcagtctgcaacctgaagattttgcaacttactactgtcagcagatgcacccgcgcgccccgaagaccttcggccaagggaccaaggtggaaatcaaa

SEQ ID NO: 168 - protein, 108 aa, Artificial Sequence
  anti-CD47 Ka3 kappa variable light domain
DIQMTQSPSSLSASVGDRVTITCRASQSISSYLNWYQQKPGKAPKLLIYAASSLQSGVPSRFSGSGSGTDFTLTISSLQPEDFATYYCQQMHPRAPKTFGQGTKVEIK

SEQ ID NO: 169 - DNA, 324 bp, Artificial Sequence
  anti-CD47 Ka3A2 kappa variable light domain
gacatccagatgacccagtctccatcctccctgtctgcatctgtaggagacagagtcaccatcacttgccgggcaagtcagagcattagtaagtatttaaattggtatcagcagaaaccagggaaagcccctaagctcctgatctatgctgcatccaggttgcaaagtggggtcccatcaaggttcagtggcagtggatctgggacagatttcactctcaccatcagcagtctgcaacctgaagattttgcaacttactactgtcagcagatgcatcctcgctcgccgaaaaccttcggccaagggaccaaggtggaaatcaaa

SEQ ID NO: 170 - protein, 108 aa, Artificial Sequence
  anti-CD47 Ka3A2 kappa variable light domain
DIQMTQSPSSLSASVGDRVTITCRASQSISKYLNWYQQKPGKAPKLLIYAASRLQSGVPSRFSGSGSGTDFTLTISSLQPEDFATYYCQQMHPRSPKTFGQGTKVEIK

SEQ ID NO: 171 - DNA, 324 bp, Artificial Sequence
  anti-CD47 Ka3H3 kappa variable light domain
gacatccagatgacccagtctccatcctccctgtctgcatctgtaggagacagagtcaccatcacttgccaggcgagtcaggacattgctaagtatttaaattggtatcagcagaaaccagggaaagcccctaagctcctgatctatgctgcatccgctttgcaaagtggggtcccatcaaggttcagtggcagtggatctgggacagatttcactctcaccatcagcagtctgcaacctgaagattttgcaacttactactgtcagcagatgcatcctcgctcgccgaaaaccttcggccaagggaccaaggtggaaatcaaa

SEQ ID NO: 172 - protein, 108 aa, Artificial Sequence
  anti-CD47 Ka3H3 kappa variable light domain
DIQMTQSPSSLSASVGDRVTITCQASQDIAKYLNWYQQKPGKAPKLLIYAASALQSGVPSRFSGSGSGTDFTLTISSLQPEDFATYYCQQMHPRSPKTFGQGTKVEIK

SEQ ID NO: 173 - DNA, 324 bp, Artificial Sequence
  anti-CD47 Ka3A3 kappa variable light domain
gacatccagatgacccagtctccatcctccctgtctgcatctgtaggagacagagtcaccatcacttgccgggcaagtcagagcattgctagttatttaaattggtatcagcagaaaccagggaaagcccctaagctcctgatctatgcggcatccaggttgcaaagtggggtcccatcaaggttcagtggcagtggatctgggacagatttcactctcaccatcagcagtctgcaacctgaagattttgcaacttactactgtcagcagatgcatcctcgcgcgccgaaaaccttcggccaagggaccaaggtggaaatcaaa

SEQ ID NO: 174 - protein, 108 aa, Artificial Sequence
  anti-CD47 Ka3A3 kappa variable light domain
DIQMTQSPSSLSASVGDRVTITCRASQSIASYLNWYQQKPGKAPKLLIYAASRLQSGVPSRFSGSGSGTDFTLTISSLQPEDFATYYCQQMHPRAPKTFGQGTKVEIK

SEQ ID NO: 175 - DNA, 324 bp, Artificial Sequence
  anti-CD47 Ka3H8 kappa variable light domain
gacatccagatgacccagtctccatcctccctgtctgcatctgtaggagacagagtcaccatcacttgccgggcaagtcagagcattgcgagttatttaaattggtatcagcagaaaccagggaaagcccctaagctcctgatctatgcggcatccaggttgcaaagtggggtcccatcaaggttcagtggcagtggatctgggacagatttcactctcaccatcagcagtctgcaacctgaagattttgcaacttactactgtcagcagatgcatcctcgctcgccgaaaaccttcggccaagggaccaaggtggaaatcaaa

SEQ ID NO: 176 - protein, 108 aa, Artificial Sequence
  anti-CD47 Ka3H8 kappa variable light domain
DIQMTQSPSSLSASVGDRVTITCRASQSIASYLNWYQQKPGKAPKLLIYAASRLQSGVPSRFSGSGSGTDFTLTISSLQPEDFATYYCQQMHPRSPKTFGQGTKVEIK

SEQ ID NO: 177 - DNA, 324 bp, Artificial Sequence
  anti-CD47 Ka3B2 kappa variable light domain
gacatccagatgacccagtctccatcctccctgtctgcatctgtaggagacagagtcaccatcacttgccgggcaagtcagaacattggtaagtatttaaattggtatcagcagaaaccagggaaagcccctaagctcctgatctatagtgcatccaggttgcaaagtggggtcccatcaaggttcagtggcagtggatctgggacagatttcactctcaccatcagcagtctgcaacctgaagattttgcaacttactactgtcagcagatgcatcctcgcgcgccgaaaaccttcggccaagggaccaaggtggaaatcaaa

SEQ ID NO: 178 - protein, 108 aa, Artificial Sequence
  anti-CD47 Ka3B2 kappa variable light domain
DIQMTQSPSSLSASVGDRVTITCRASQNIGKYLNWYQQKPGKAPKLLIYSASRLQSGVPSRFSGSGSGTDFTLTISSLQPEDFATYYCQQMHPRAPKTFGQGTKVEIK

SEQ ID NO: 179 - DNA, 324 bp, Artificial Sequence
  anti-CD47 Ka3C5 kappa variable light domain
gacatccagatgacccagtctccatcctccctgtctgcatctgtaggagacagagtcaccatcacttgccgggcaagtcagagcattagtaggtatttaaattggtatcagcagaaaccagggaaagcccctaagctcctgatctattctgcatcctctttgcaaagtggggtcccatcaaggttcagtggcagtggatctgggacagatttcactctcaccatcagcagtctgcaacctgaagattttgcaacttactactgtcagcagatgcatcctcgcgccccgaaaaccttcggccaagggaccaaggtggaaatcaaa

SEQ ID NO: 180 - protein, 108 aa, Artificial Sequence
  anti-CD47 Ka3C5 kappa variable light domain
DIQMTQSPSSLSASVGDRVTITCRASQSISRYLNWYQQKPGKAPKLLIYSASSLQSGVPSRFSGSGSGTDFTLTISSLQPEDFATYYCQQMHPRAPKTFGQGTKVEIK

SEQ ID NO: 181 - DNA, 324 bp, Artificial Sequence
  anti-CD47 Ka3G2 kappa variable light domain
gacatccagatgacccagtctccatcctccctgtctgcatctgtaggagacagagtcaccatcacttgccgggcaagtcagagcattgataagtatttaaattggtatcagcagaaaccagggaaagcccctaagctcctgatctatgctgcatccaggttgcaaagtggggtcccatcaaggttcagtggcagtggatctgggacagatttcactctcaccatcagcagtctgcaacctgaagattttgcaacttactactgtcagcagatgcatcctcgcgggccgaaaaccttcggccaagggaccaaggtggaaatcaaa

SEQ ID NO: 182 - protein, 108 aa, Artificial Sequence
  anti-CD47 Ka3G2 kappa variable light domain
DIQMTQSPSSLSASVGDRVTITCRASQSIDKYLNWYQQKPGKAPKLLIYAASRLQSGVPSRFSGSGSGTDFTLTISSLQPEDFATYYCQQMHPRGPKTFGQGTKVEIK

SEQ ID NO: 183 - DNA, 324 bp, Artificial Sequence
  anti-CD47 Ka3D3 kappa variable light domain
gacatccagatgacccagtctccatcctccctgtctgcatctgtaggagacagagtcaccatcacttgccgggcaagtcagagcattggtaagtatttaaattggtatcagcagaaaccagggaaagcccctaagctcctgatctatgctgcatccaggttgcaaagtggggtcccatcaaggttcagtggcagtggatctgggacagatttcactctcaccatcagcagtctgcaacctgaagattttgcaacttactactgtcagcagatgcatcctcgcgcgccgaaaaccttcggccaagggaccaaggtggaaatcaaa

SEQ ID NO: 184 - protein, 108 aa, Artificial Sequence
  anti-CD47 Ka3D3 kappa variable light domain
DIQMTQSPSSLSASVGDRVTITCRASQSIGKYLNWYQQKPGKAPKLLIYAASRLQSGVPSRFSGSGSGTDFTLTISSLQPEDFATYYCQQMHPRAPKTFGQGTKVEIK

SEQ ID NO: 185 - DNA, 333 bp, Artificial Sequence
  anti-CD47 Kc4 kappa variable light domain
cagtctgccctgactcagcctgcctccgtgtctgggtctcctggacagtcgatcaccatctcctgcactggaaccagcagtgacgttggtggttataactatgtctcctggtaccaacagcacccaggcaaagcccccaaactcatgatttatgaggtcagtaatcggccctcaggggtttctaatcgcttctctggctccaagtctggcaacacggcctccctgaccatctctgggctccaggctgaggacgaggctgattattactgcagctcatatgattggtggttccgccccaaggtgttcggcggagggaccaagctgaccgtccta

SEQ ID NO: 186 - protein, 111 aa, Artificial Sequence
  anti-CD47 Kc4 kappa variable light domain
QSALTQPASVSGSPGQSITISCTGTSSDVGGYNYVSWYQQHPGKAPKLMIYEVSNRPSGVSNRFSGSKSGNTASLTISGLQAEDEADYYCSSYDWWFRPKVFGGGTKLTVL

SEQ ID NO: 187 - DNA, 333 bp, Artificial Sequence
  anti-CD47 Kc4G11 kappa variable light domain
cagtctgccctgactcagcctgcctccgtgtctgggtctcctggacagtcgatcaccatctcctgcactggaaccagcagtgacgttgggaaggcgaactatgtctcctggtaccaacagcacccaggcaaagcccccaaactcatgatttataaggatagtgatcggccctcaggggtttctaatcgcttctctggctccaagtctggcaacacggcctccctgaccatctctgggctccaggctgaggacgaggctgattattactgcagctcatatgattggtggttccgccccaaggtgttcggcggagggaccaagctgaccgtccta

SEQ ID NO: 188 - protein, 111 aa, Artificial Sequence
  anti-CD47 Kc4G11 kappa variable light domain
QSALTQPASVSGSPGQSITISCTGTSSDVGKANYVSWYQQHPGKAPKLMIYKDSDRPSGVSNRFSGSKSGNTASLTISGLQAEDEADYYCSSYDWWFRPKVFGGGTKLTVL

SEQ ID NO: 189 - DNA, 333 bp, Artificial Sequence
  anti-CD47 Kc4C11 kappa variable light domain
cagtctgccctgactcagcctgcctccgtgtctgggtctcctggacagtcgatcaccatctcctgcactggaaccagcagtgacgttagggggaataactatgtctcctggtaccaacagcacccaggcaaagcccccaaactcatgatttatgagaatagtaagcggccctcaggggtttctaatcgcttctctggctccaagtctggcaacacggcctccctgaccatctctgggctccaggctgaggacgaggctgattattactgcagctcatatgattggtggttccgccccaaggtgttcggcggagggaccaagctgaccgtccta

SEQ ID NO: 190 - protein, 111 aa, Artificial Sequence
  anti-CD47 Kc4C11 kappa variable light domain
QSALTQPASVSGSPGQSITISCTGTSSDVRGNNYVSWYQQHPGKAPKLMIYENSKRPSGVSNRFSGSKSGNTASLTISGLQAEDEADYYCSSYDWWFRPKVFGGGTKLTVL

SEQ ID NO: 191 - DNA, 333 bp, Artificial Sequence
  anti-CD47 Kc4A1 kappa variable light domain
cagtctgccctgactcagcctgcctccgtgtctgggtctcctggacagtcgatcaccatctcctgcactggaaccagcagtgacgttagtgcgaggaactatgtctcctggtaccaacagcacccaggcaaagcccccaaactcatgatttatgagagtagtaagcggccctcaggggtttctaatcgcttctctggctccaagtctggcaacacggcctccctgaccatctctgggctccaggctgaggacgaggctgattattactgcagctcatatgattggtggttccgccccaaggtgttcggcggagggaccaagctgaccgtccta

SEQ ID NO: 192 - protein, 111 aa, Artificial Sequence
  anti-CD47 Kc4A1 kappa variable light domain
QSALTQPASVSGSPGQSITISCTGTSSDVSARNYVSWYQQHPGKAPKLMIYESSKRPSGVSNRFSGSKSGNTASLTISGLQAEDEADYYCSSYDWWFRPKVFGGGTKLTVL

SEQ ID NO: 193 - DNA, 333 bp, Artificial Sequence
  anti-CD47 Kc4A4 kappa variable light domain
cagtctgccctgactcagcctgcctccgtgtctgggtctcctggacagtcgatcaccatctcctgcactagaaccagcagtgacgttaataatactaactatgtctcctggtaccaacagcacccaggcaaagcccccaaactcatgatttataagactagtggtcggccctcaggggtttctaatcgcttctctggctccaagtctggcaacacggcctccctgaccatctctgggctccaggctgaggacgaggctgattattactgcagctcatatgattggtggttccgccccaaggtgttcggcggagggaccaagctgaccgtccta

SEQ ID NO: 194 - protein, 111 aa, Artificial Sequence
  anti-CD47 Kc4A4 kappa variable light domain
QSALTQPASVSGSPGQSITISCTRTSSDVNNTNYVSWYQQHPGKAPKLMIYKTSGRPSGVSNRFSGSKSGNTASLTISGLQAEDEADYYCSSYDWWFRPKVFGGGTKLTVL

SEQ ID NO: 195 - DNA, 333 bp, Artificial Sequence
  anti-CD47 Kc4E10 kappa variable light domain
cagtctgccctgactcagcctgcctccgtgtctgggtctcctggacagtcgatcaccatctcctgcactggaaccagcagtgacgttaattctgctaactatgtctcctggtaccaacagcacccaggcaaagcccccaaactcatgatttataagagtagtagtcggccctcaggggtttctaatcgcttctctggctccaagtctggcaacacggcctccctgaccatctctgggctccaggctgaggacgaggctgattattactgcagctcatatgattggtggttccgccccaaggtgttcggcggagggaccaagctgaccgtccta

SEQ ID NO: 196 - protein, 111 aa, Artificial Sequence
  anti-CD47 Kc4E10 kappa variable light domain
QSALTQPASVSGSPGQSITISCTGTSSDVNSANYVSWYQQHPGKAPKLMIYKSSSRPSGVSNRFSGSKSGNTASLTISGLQAEDEADYYCSSYDWWFRPKVFGGGTKLTVL

SEQ ID NO: 197 - DNA, 333 bp, Artificial Sequence
  anti-CD47 Kc4G9 kappa variable light domain
cagtctgccctgactcagcctgcctccgtgtccgggtctcctggacagtcgatcaccatctcctgcactggaaccagcagtgacgttgagaggaagaactatgtctcctggtaccaacagcacccaggcaaagcccccaaactcatgatttataagaatagtactcggccctcaggggtttctaatcgcttctctggctccaagtctggcaacacggcctccctgaccatctctgggctccaggctgaggacgaggctgattattactgcagctcatatgattggtggttccgccccaaggtgttcggcggagggaccaagctgaccgtccta

SEQ ID NO: 198 - protein, 111 aa, Artificial Sequence
  anti-CD47 Kc4G9 kappa variable light domain
QSALTQPASVSGSPGQSITISCTGTSSDVERKNYVSWYQQHPGKAPKLMIYKNSTRPSGVSNRFSGSKSGNTASLTISGLQAEDEADYYCSSYDWWFRPKVFGGGTKLTVL

SEQ ID NO: 199 - DNA, 333 bp, Artificial Sequence
  anti-CD47 Kc4C3 kappa variable light domain
cagtctgccctgactcagcctgcctccgtgtctgggtctcctggacagtcgatcaccatctcctgcactggaaccagcagtgacgttagggcggctaactatgtctcctggtaccaacagcacccaggcaaagcccccaaactcatgatttataagaatagtactcggccctcaggggtttctaatcgcttctctggctccaagtctggcaacacggcctccctgaccatctctgggctccaggctgaggacgaggctgattattactgcagctcatatgattggtggttccgccccaaggtgttcggcggagggaccaagctgaccgtccta

SEQ ID NO: 200 - protein, 111 aa, Artificial Sequence
  anti-CD47 Kc4C3 kappa variable light domain
QSALTQPASVSGSPGQSITISCTGTSSDVRAANYVSWYQQHPGKAPKLMIYKNSTRPSGVSNRFSGSKSGNTASLTISGLQAEDEADYYCSSYDWWFRPKVFGGGTKLTVL

SEQ ID NO: 201 - DNA, 333 bp, Artificial Sequence
  anti-CD47 Kc4F4 kappa variable light domain
cagtctgccctgactcagcctgcctccgtgtctgggtctcctggacagtcgatcaccatctcctgcactggaaccagcagtgacgttaggagggctaactatgtctcctggtaccaacagcacccaggcaaagcccccaaactcatgatttatcaggatagtagtcggccctcaggggtttctaatcgcttctctggctccaagtctggcaacacggcctccctgaccatctctgggctccaggctgaggacgaggctgattattactgcagctcatatgattggtggttccgccccaaggtgttcggcggagggaccaagctgaccgtccta

SEQ ID NO: 202 - protein, 111 aa, Artificial Sequence
  anti-CD47 Kc4F4 kappa variable light domain
QSALTQPASVSGSPGQSITISCTGTSSDVRRANYVSWYQQHPGKAPKLMIYQDSSRPSGVSNRFSGSKSGNTASLTISGLQAEDEADYYCSSYDWWFRPKVFGGGTKLTVL

SEQ ID NO: 203 - DNA, 333 bp, Artificial Sequence
  anti-CD47 Kc4B1 kappa variable light domain
cagtctgccctgactcagcctgcctccgtgtctgggtctcctggacagtcgatcaccatctcctgcactggaaccagcagtgacgttagggctaataactatgtctcctggtaccaacagcacccaggcaaagcccccaaactcatgatttatgagagtagtgcgcggccctcaggggtttctaatcgcttctctggctccaagtctggcaacacggcctccctgaccatctctgggctccaggctgaggacgaggctgattattactgcagctcatatgattggtggttccgccccaaggtgttcggcggagggaccaagctgaccgtccta

SEQ ID NO: 204 - protein, 111 aa, Artificial Sequence
  anti-CD47 Kc4B1 kappa variable light domain
QSALTQPASVSGSPGQSITISCTGTSSDVRANNYVSWYQQHPGKAPKLMIYESSARPSGVSNRFSGSKSGNTASLTISGLQAEDEADYYCSSYDWWFRPKVFGGGTKLTVL

SEQ ID NO: 205 - DNA, 333 bp, Artificial Sequence
  anti-CD47 Kc4E2 kappa variable light domain
cagtctgccctgactcagcctgcctccgtgtctgggtctcctggacagtcgatcaccatctcctgcactggaaccagcagtgacgtttattataataagtatgtctcctggtaccaacagcacccaggcaaagcccccaaactcatgatttatgagagtagtaagcggccctcaggggtttctaatcgcttctctggctccaagtctggcaacacggcctccctgaccatctctgggctccaggctgaggacgaggctgattattactgcagctcatatgattggtggttccgccccaaggtgttcggcggagggaccaagctgaccgtccta

SEQ ID NO: 206 - protein, 111 aa, Artificial Sequence
  anti-CD47 Kc4E2 kappa variable light domain
QSALTQPASVSGSPGQSITISCTGTSSDVYYNKYVSWYQQHPGKAPKLMIYESSKRPSGVSNRFSGSKSGNTASLTISGLQAEDEADYYCSSYDWWFRPKVFGGGTKLTVL

SEQ ID NO: 207 - DNA, 336 bp, Artificial Sequence
  anti-CD19 C2 lambda variable light domain
aattttatgctgactcagccccactctgtgtcggagtctccggggaagacggtaaccatctcctgcacccgcagcagtggctctatcgaagataagtatgtgcagtggtaccagcagcgcccgggcagttcccccaccattgtgatctattatgataacgaaagaccctctggggtccctgatcggttctctggctccatcgacagctcctccaactctgcctccctcaccatctctggactgaagactgaggacgaggctgactactactgtcagacctacgaccagagcctgtatggttgggtgttcggcggagggaccaagctgaccgtccta

SEQ ID NO: 208 - protein, 112 aa, Artificial Sequence
  anti-CD19 C2 lambda variable light domain
NFMLTQPHSVSESPGKTVTISCTRSSGSIEDKYVQWYQQRPGSSPTIVIYYDNERPSGVPDRFSGSIDSSSNSASLTISGLKTEDEADYYCQTYDQSLYGWVFGGGTKLTVL

SEQ ID NO: 209 - DNA, 336 bp, Artificial Sequence
  anti-CD19 A6 lambda variable light domain
aattttatgctgactcagccccactctgtgtcggagtctccggggaagacggtaaccatctcctgcacccgcagcagtggctctatcggtgataagtatgtgcagtggtaccagcagcgcccgggcagttcccccaccattgtgatctattatgataacgaaagaccctctggggtccctgatcggttctctggctccatcgacagctcctccaactctgcctccctcaccatctctggactgaagactgaggacgaggctgactactactgtcagacgtacgacgagagcctgtatggttgggtgttcggcggagggaccaagctgaccgtccta

SEQ ID NO: 210 - protein, 112 aa, Artificial Sequence
  anti-CD19 A6 lambda variable light domain
NFMLTQPHSVSESPGKTVTISCTRSSGSIGDKYVQWYQQRPGSSPTIVIYYDNERPSGVPDRFSGSIDSSSNSASLTISGLKTEDEADYYCQTYDESLYGWVFGGGTKLTVL

SEQ ID NO: 211 - DNA, 336 bp, Artificial Sequence
  anti-CD19 C6 lambda variable light domain
aattttatgctgactcagccccactctgtgtcggagtctccggggaagacggtaaccatctcctgcacccgcagcagtggctctatcaatgataagtatgtgcagtggtaccagcagcgcccgggcagttcccccaccattgtgatctattttgataacgaaagaccctctggggtccctgatcggttctctggctccatcgacagctcctccaactctgcctccctcaccatctctggactgaagactgaggacgaggctgactactactgtcagacctacgacaccagcctgtatggttgggtgttcggcggagggaccaagctgaccgtccta

SEQ ID NO: 212 - protein, 112 aa, Artificial Sequence
  anti-CD19 C6 lambda variable light domain
NFMLTQPHSVSESPGKTVTISCTRSSGSINDKYVQWYQQRPGSSPTIVIYFDNERPSGVPDRFSGSIDSSSNSASLTISGLKTEDEADYYCQTYDTSLYGWVFGGGTKLTVL

SEQ ID NO: 213 - DNA, 336 bp, Artificial Sequence
  anti-CD19 C9 lambda variable light domain
aattttatgctgactcagccccactctgtgtcggagtctccggggaagacggtaaccatctcctgcacccgcagcagtggctctatcgctgataagtatgtgcagtggtaccagcagcgcccgggcagttcccccaccattgtgatctattatgataacgaaagaccctctggggtccctgatcggttctctggctccatcgacagctcctccaactctgcctccctcaccatctctggactgaagactgaggacgaggctgactactactgtcagacctacgacgagagcctgtatggttgggtgttcggcggagggaccaagctgaccgtccta

SEQ ID NO: 214 - protein, 112 aa, Artificial Sequence
  anti-CD19 C9 lambda variable light domain
NFMLTQPHSVSESPGKTVTISCTRSSGSIADKYVQWYQQRPGSSPTIVIYYDNERPSGVPDRFSGSIDSSSNSASLTISGLKTEDEADYYCQTYDESLYGWVFGGGTKLTVL

SEQ ID NO: 215 - DNA, 336 bp, Artificial Sequence
  anti-CD19 B11 lambda variable light domain
aattttatgctgactcagccccactctgtgtcggagtctccggggaagacggtaaccatctcctgcacccgcagcagtggctctatcgaagataagtatgtgcagtggtaccagcagcgcccgggcagttcccccaccattgtgatctattatgataacgaaagaccctctggggtccctgatcggttctctggctccatcgacagctcctccaactctgcctccctcaccatctctggactgaagactgaggacgaggctgactactactgtcagacctacgacaacagcctgtatggttgggtgttcggcggagggaccaagctgaccgtccta

SEQ ID NO: 216 - protein, 112 aa, Artificial Sequence
  anti-CD19 B11 lambda variable light domain
NFMLTQPHSVSESPGKTVTISCTRSSGSIEDKYVQWYQQRPGSSPTIVIYYDNERPSGVPDRFSGSIDSSSNSASLTISGLKTEDEADYYCQTYDNSLYGWVFGGGTKLTVL

SEQ ID NO: 217 - DNA, 336 bp, Artificial Sequence
  anti-CD19 D11 lambda variable light domain
aattttatgctgactcagccccactctgtgtcggagtctccggggaagacggtaaccatctcctgcacccgcagcagtggcagcatcgatgataagtttgtgcagtggtaccagcagcgcccgggcagttcccccaccactgtgatctattatgataacattagaccctctggggtccctgatcggttctctggctccatcgacagctcctccaactctgcctccctcaccatctctggactgaagactgaggacgaggctgactactactgtcagtcctatgacgcgagcctgtatggttgggtgttcggcggagggaccaagctgaccgtccta

SEQ ID NO: 218 - protein, 112 aa, Artificial Sequence
  anti-CD19 D11 lambda variable light domain
NFMLTQPHSVSESPGKTVTISCTRSSGSIDDKFVQWYQQRPGSSPTTVIYYDNIRPSGVPDRFSGSIDSSSNSASLTISGLKTEDEADYYCQSYDASLYGWVFGGGTKLTVL

SEQ ID NO: 219 - DNA, 336 bp, Artificial Sequence
  anti-CD19 B7 lambda variable light domain
aattttatgctgactcagccccactctgtgtcggagtctccggggaagacggtaaccatctcctgcacccgcagcagtggctctatcgcggataagtatgtgcagtggtaccagcagcgcccgggcagttcccccaccactgtgatctatgaggataaccaaagaccctctggggtccctgatcggttctctggctccatcgacagctcctccaactctgcctccctcaccatctctggactgaagactgaggacgaggctgactactactgtcagtcctatgacagcagcctgtatggttgggtgttcggcggagggaccaagctgaccgtccta

SEQ ID NO: 220 - protein, 112 aa, Artificial Sequence
  anti-CD19 B7 lambda variable light domain
NFMLTQPHSVSESPGKTVTISCTRSSGSIADKYVQWYQQRPGSSPTTVIYEDNQRPSGVPDRFSGSIDSSSNSASLTISGLKTEDEADYYCQSYDSSLYGWVFGGGTKLTVL

SEQ ID NO: 221 - DNA, 330 bp, Artificial Sequence
  dummy variable light domain 1
cagtctgtgttgacgcagccgccctcagtgtctgcggccccaggacagaaggtcaccatctcctgctctggaagcagctccaatattgagactggttctgtatcctggtaccagcagctcccaggaacagcccccaaactcctcatttatgacaataataagcgaccctcagggattcctgaccgattctctggctccaagtctggcacgtcagccaccctgggcatcaccggactccagactggggacgaggccgattattactgcggaacatgggatgacagcctgcctggatgggtgttcggcggagggaccaagctgaccgtccta

SEQ ID NO: 222 - protein, 110 aa, Artificial Sequence
  dummy variable light domain 1
QSVLTQPPSVSAAPGQKVTISCSGSSSNIETGSVSWYQQLPGTAPKLLIYDNNKRPSGIPDRFSGSKSGTSATLGITGLQTGDEADYYCGTWDDSLPGWVFGGGTKLTVL

SEQ ID NO: 223 - DNA, 333 bp, Artificial Sequence
  dummy variable light domain 2
gaaatagtgatgacgcagtctccagccaccctgtctgtgtctccaggggaaagagccaccctctcctgcagggccagtcagacggttaagaataatttagcctggtaccagcagaaacctggccaggctcccaggctcctcatctatggtgcatccaccagggccactggtatcccagccaggttcagtggcagtgggtctgggacagagttcactctcaccatcagcagcctgcagtctgaagattttgcagtttattactgtcagcagtataacaactggttgcccatcaacccctataccttcggccaagggaccaaggtggaaatcaaa

SEQ ID NO: 224 - protein, 111 aa, Artificial Sequence
  dummy variable light domain 2
EIVMTQSPATLSVSPGERATLSCRASQTVKNNLAWYQQKPGQAPRLLIYGASTRATGIPARFSGSGSGTEFTLTISSLQSEDFAVYYCQQYNNWLPINPYTFGQGTKVEIK

SEQ ID NO: 225 - protein, 8 aa, Artificial Sequence
  anti-CD47 heavy chain CDHR1
GFTFSSYA

SEQ ID NO: 226 - protein, 8 aa, Artificial Sequence
  anti-CD47 heavy chain CDHR2
ISGSGGST

SEQ ID NO: 227 - protein, 9 aa, Artificial Sequence
  anti-CD47 heavy chain CDHR3
AKSYGAFDY

SEQ ID NO: 228 - protein, 6 aa, Artificial Sequence
  anti-CD47 kappa light chain CDRL1
QDINKY

SEQ ID NO: 229 - protein, 6 aa, Artificial Sequence
  anti-CD47 kappa light chain CDRL1
QDINRY

SEQ ID NO: 230 - protein, 6 aa, Artificial Sequence
  anti-CD47 kappa light chain CDRL1
QNIGKY

SEQ ID NO: 231 - protein, 6 aa, Artificial Sequence
  anti-CD47 kappa light chain CDRL1
QSIARY

SEQ ID NO: 232 - protein, 6 aa, Artificial Sequence
  anti-CD47 kappa light chain CDRL1
QSIASY

SEQ ID NO: 233 - protein, 6 aa, Artificial Sequence
  anti-CD47 kappa light chain CDRL1
QSIDKY

SEQ ID NO: 234 - protein, 6 aa, Artificial Sequence
  anti-CD47 kappa light chain CDRL1
QSIDRY

SEQ ID NO: 235 - protein, 6 aa, Artificial Sequence
  anti-CD47 kappa light chain CDRL1
QSIGKY

SEQ ID NO: 236 - protein, 6 aa, Artificial Sequence
  anti-CD47 kappa light chain CDRL1
QSIGRY

SEQ ID NO: 237 - protein, 6 aa, Artificial Sequence
  anti-CD47 kappa light chain CDRL1
QSINRY

SEQ ID NO: 238 - protein, 6 aa, Artificial Sequence
  anti-CD47 kappa light chain CDRL1
QSISKY

SEQ ID NO: 239 - protein, 6 aa, Artificial Sequence
  anti-CD47 kappa light chain CDRL1
QSISRY

SEQ ID NO: 240 - protein, 6 aa, Artificial Sequence
  anti-CD47 kappa light chain CDRL1
QSISSY

SEQ ID NO: 241 - protein, 6 aa, Artificial Sequence
  anti-CD47 kappa light chain CDRL1
QSIAKY

SEQ ID NO: 242 - protein, 3 aa, Artificial Sequence
  anti-CD47 kappa light chain CDRL2
AAS

SEQ ID NO: 243 - protein, 3 aa, Artificial Sequence
  anti-CD47 kappa light chain CDRL2
GAS

SEQ ID NO: 244 - protein, 3 aa, Artificial Sequence
  anti-CD47 kappa light chain CDRL2
NAS

SEQ ID NO: 245 - protein, 3 aa, Artificial Sequence
  anti-CD47 kappa light chain CDRL2
SAS

SEQ ID NO: 246 - protein, 10 aa, Artificial Sequence
  anti-CD47 kappa light chain CDRL3
QQKHPRGPRT

SEQ ID NO: 247 - protein, 10 aa, Artificial Sequence
  anti-CD47 kappa light chain CDRL3
QQFHKRAPQT

SEQ ID NO: 248 - protein, 10 aa, Artificial Sequence
  anti-CD47 kappa light chain CDRL3
QQFHKRRPQT

SEQ ID NO: 249 - protein, 10 aa, Artificial Sequence
  anti-CD47 kappa light chain CDRL3
QQFHKRSPQT

SEQ ID NO: 250 - protein, 10 aa, Artificial Sequence
  anti-CD47 kappa light chain CDRL3
QQKHPRAPRT

SEQ ID NO: 251 - protein, 10 aa, Artificial Sequence
  anti-CD47 kappa light chain CDRL3
QQKHPRSPRT

SEQ ID NO: 252 - protein, 10 aa, Artificial Sequence
  anti-CD47 kappa light chain CDRL3
QQKHPRYPRT

SEQ ID NO: 253 - protein, 10 aa, Artificial Sequence
  anti-CD47 kappa light chain CDRL3
QQKHPRNPRT

SEQ ID NO: 254 - protein, 10 aa, Artificial Sequence
  anti-CD47 kappa light chain CDRL3
QQMHPRAPKT

SEQ ID NO: 255 - protein, 10 aa, Artificial Sequence
  anti-CD47 kappa light chain CDRL3
QQMHPRGPKT

SEQ ID NO: 256 - protein, 10 aa, Artificial Sequence
  anti-CD47 kappa light chain CDRL3
QQMHPRSPKT

SEQ ID NO: 257 - protein, 10 aa, Artificial Sequence
  anti-CD47 kappa light chain CDRL3
QQRHPRAPRT

SEQ ID NO: 258 - protein, 10 aa, Artificial Sequence
  anti-CD47 kappa light chain CDRL3
QQRHKRSPQT

SEQ ID NO: 259 - protein, 10 aa, Artificial Sequence
  anti-CD47 kappa light chain CDRL3
QQRHPRGPRT

SEQ ID NO: 260 - protein, 10 aa, Artificial Sequence
  anti-CD47 kappa light chain CDRL3
QQRHPRGPST

SEQ ID NO: 261 - protein, 10 aa, Artificial Sequence
  anti-CD47 kappa light chain CDRL3
QQRHPRGPTT

SEQ ID NO: 262 - protein, 9 aa, Artificial Sequence
  anti-CD47 lambda light chain CDRL1
SSDVGGYNY

SEQ ID NO: 263 - protein, 9 aa, Artificial Sequence
  anti-CD47 lambda light chain CDRL1
SSDVERKNY

SEQ ID NO: 264 - protein, 9 aa, Artificial Sequence
  anti-CD47 lambda light chain CDRL1
SSDVRANNY

SEQ ID NO: 265 - protein, 9 aa, Artificial Sequence
  anti-CD47 lambda light chain CDRL1
SSDVYYNKY

SEQ ID NO: 266 - protein, 9 aa, Artificial Sequence
  anti-CD47 lambda light chain CDRL1
SSDVGKANY

SEQ ID NO: 267 - protein, 9 aa, Artificial Sequence
  anti-CD47 lambda light chain CDRL1
SSDVRGNNY

SEQ ID NO: 268 - protein, 9 aa, Artificial Sequence
  anti-CD47 lambda light chain CDRL1
SSDVSARNY

SEQ ID NO: 269 - protein, 9 aa, Artificial Sequence
  anti-CD47 lambda light chain CDRL1
SSDVNSANY

SEQ ID NO: 270 - protein, 9 aa, Artificial Sequence
  anti-CD47 lambda light chain CDRL1
SSDVRAANY

SEQ ID NO: 271 - protein, 9 aa, Artificial Sequence
  anti-CD47 lambda light chain CDRL1
SSDVRRANY

SEQ ID NO: 272 - protein, 9 aa, Artificial Sequence
  anti-CD47 lambda light chain CDRL1
SSDVNNTNY

SEQ ID NO: 273 - protein, 3 aa, Artificial Sequence
  anti-CD47 lambda light chain CDRL2
ENS

SEQ ID NO: 274 - protein, 3 aa, Artificial Sequence
  anti-CD47 lambda light chain CDRL2
ESS

SEQ ID NO: 275 - protein, 3 aa, Artificial Sequence
  anti-CD47 lambda light chain CDRL2
EVS

SEQ ID NO: 276 - protein, 3 aa, Artificial Sequence
  anti-CD47 lambda light chain CDRL2
KDS

SEQ ID NO: 277 - protein, 3 aa, Artificial Sequence
  anti-CD47 lambda light chain CDRL2
KNS

SEQ ID NO: 278 - protein, 3 aa, Artificial Sequence
  anti-CD47 lambda light chain CDRL2
KSS

SEQ ID NO: 279 - protein, 3 aa, Artificial Sequence
  anti-CD47 lambda light chain CDRL2
KTS

SEQ ID NO: 280 - protein, 3 aa, Artificial Sequence
  anti-CD47 lambda light chain CDRL2
QDS

SEQ ID NO: 281 - protein, 11 aa, Artificial Sequence
  anti-CD47 lambda light chain CDRL3
SSYDWWFRPKV

SEQ ID NO: 282 - protein, 94 aa, Homo sapiens
DIQMTQSPSSLSASVGDRVTITCQASQDISNYLNWYQQKPGKAPKLLIYDASNLETGVPSRFSGSGSGTDFTFTISSLQPEDIATYYCQYDNLP

SEQ ID NO: 283 - DNA, 21 bp, Artificial Sequence
  pNDS1 mycseq primer
ctcttctgagatgagtttttg

SEQ ID NO: 284 - DNA, 30 bp, Artificial Sequence
  pNDS1 gene3leader primer
ttattattcgcaattcctttagttgttcct

SEQ ID NO: 285 - protein, 110 aa, Artificial Sequence
  5A3-VL
DIQMTQSPSSLSASVGDRVTITCQASQDINKYLNWYQQKPGKAPKLLIYGASRLETGVPSRFSGSGSGTDFTFTISSLQPEDIATYYCQQKHPRGPRTFGQGTKVEIKRT

SEQ ID NO: 286 - protein, 110 aa, Artificial Sequence
  5A3-M3-VL
DIQMTQSPSSLSASVGDRVTITCQASQSISSYLNWYQQKPGKAPKLLIYAASSLETGVPSRFSGSGSGTDFTFTISSLQPEDIATYYCQQKHPRGPRTFGQGTKVEIKRT

SEQ ID NO: 287 - protein, 110 aa, Artificial Sequence
  5A3-M5-VL
DIQMTQSPSSLSASVGDRVTITCQASQDINKYLNWYQQKPGKAPKLLIYGASRLETGVPSRFSGSGSGTDFTFTISSLQPEDIATYYCQQKHPRYPRTFGQGTKVEIKRT